European Patent Specification EP 2 968 583 B1, published June 4, 2025. Title: Method of producing an immunoligand/payload conjugate. Applicant: NBE Therapeutics. The sequence listing filed with the application follows.

SEQUENCE LISTING (58 sequences)

SEQ ID NO: 1 - DNA, 417 bp, Artificial Sequence
  VH coding region of humanized anti-human CD19 antibody hBU12
atgggatggagctggatctttcttttcctcctgtcaggaactgcaggtgtccattgtcaggttcagctgcaagagtctggccctgggttggttaagccctcccagaccctcagtctgacttgtactgtgtctgggggttcaatcagcacttctggtatgggtgtaggctggattaggcagcacccagggaagggtctggagtggattggacacatttggtgggatgatgacaagagatataacccagccctgaagagcagagtgacaatctctgtggatacctccaagaaccagtttagcctcaagctgtccagtgtgacagctgcagatactgctgtctactactgtgctagaatggaactttggtcctactattttgactactggggccaaggcacccttgtcacagtctcctca

SEQ ID NO: 2 - protein, 139 aa, Artificial Sequence
  amino acid sequence of VH region of humanized anti-human CD19 antibody hBU12
MGWSWIFLFLLSGTAGVHCQVQLQESGPGLVKPSQTLSLTCTVSGGSISTSGMGVGWIRQHPGKGLEWIGHIWWDDDKRYNPALKSRVTISVDTSKNQFSLKLSSVTAADTAVYYCARMELWSYYFDYWGQGTLVTVSS

SEQ ID NO: 3 - DNA, 375 bp, Artificial Sequence
  VL coding region of humanized anti-human CD19 antibody hBU12
atgaagttgcctgttaggctgttggtgctgatgttctggattcctgcttccagcagtgaaattgttctcacccagtctccagcaaccctgtctctctctccaggggaaagggctaccctgagctgcagtgccagctcaagtgtaagttacatgcactggtaccagcagaagccagggcaggctcccagactcctgatttatgacacatccaaactggcttctggtattccagcaaggttcagtggcagtgggtctggaacagattttacactcacaatcagcagcctggagccagaggatgttgctgtctattactgttttcaggggagtgtatacccattcacttttggccaagggacaaagttggaaatcaaa

SEQ ID NO: 4 - protein, 125 aa, Artificial Sequence
  amino acid sequence of VL region of humanized anti-human CD19 antibody hBU12
MKLPVRLLVLMFWIPASSSEIVLTQSPATLSLSPGERATLSCSASSSVSYMHWYQQKPGQAPRLLIYDTSKLASGIPARFSGSGSGTDFTLTISSLEPEDVAVYYCFQGSVYPFTFGQGTKLEIK

SEQ ID NO: 5 - DNA, 1083 bp, Artificial Sequence
  human IgG1 heavy chain constant coding region with in-frame 3' extension encoding an LPETG sortase tag, an 6xHis tag and a strepII tag
agcaccaagggcccatctgtcttccccctggcaccctcctccaagagcacctctgggggcacagctgccctgggctgcctggtcaaggactacttccctgaacctgtgacagtgtcctggaactcaggcgccctgaccagcggcgtgcacaccttcccggctgtcctacagtcctcaggactctactccctcagcagcgtggtgaccgtgccctccagcagcttgggcacccagacctacatctgcaacgtgaatcacaagcccagcaacaccaaggtggacaagaaagttgagcccaaatcttgtgacaaaactcacacatgcccaccgtgcccagcacctgaactcctggggggaccgtcagtcttcctcttccccccaaaacccaaggacaccctcatgatctcccggacccctgaggtcacatgcgtggtggtggacgtgagccacgaagaccctgaggtcaagttcaactggtacgtggacggcgtggaggtgcataatgccaagacaaagccgcgggaggagcagtacaacagcacgtaccgtgtggtcagcgtcctcaccgtcctgcaccaggactggctgaatggcaaggagtacaagtgcaaggtctccaacaaagccctcccagcccccatcgagaaaaccatctccaaagccaaagggcagccccgagaaccacaggtgtacaccctgcccccatcccgggatgagctgaccaagaaccaggtcagcctgacctgcctggtcaaaggcttctatcccagcgacatcgccgtggagtgggagagcaatgggcagccggagaacaactacaagaccacgcctcccgtgctggactccgacggctccttcttcctctacagcaagctcaccgtggacaagagcaggtggcagcaggggaacgtcttctcatgctccgtgatgcatgaggctctgcacaaccactacacacagaagagcctctccctgtctccgggtaaactgcccgagaccggccaccaccaccaccaccacggcgagcagaagctgatcagcgaggaggacctgggctggagccacccccagttcgagaagtag

SEQ ID NO: 6 - protein, 360 aa, Artificial Sequence
  amino acid sequence of human IgG1 heavy chain constant region with LPETG sortase tag, an 6xHis tag and a strepII tag
STKGPSVFPLAPSSKSTSGGTAALGCLVKDYFPEPVTVSWNSGALTSGVHTFPAVLQSSGLYSLSSVVTVPSSSLGTQTYICNVNHKPSNTKVDKKVEPKSCDKTHTCPPCPAPELLGGPSVFLFPPKPKDTLMISRTPEVTCVVVDVSHEDPEVKFNWYVDGVEVHNAKTKPREEQYNSTYRVVSVLTVLHQDWLNGKEYKCKVSNKALPAPIEKTISKAKGQPREPQVYTLPPSRDELTKNQVSLTCLVKGFYPSDIAVEWESNGQPENNYKTTPPVLDSDGSFFLYSKLTVDKSRWQQGNVFSCSVMHEALHNHYTQKSLSLSPGKLPETGHHHHHHGEQKLISEEDLGWSHPQFEK

SEQ ID NO: 7 - DNA, 414 bp, Artificial Sequence
  human IgG1 kappa light chain constant coding region with in-frame 3' extension encoding an LPETG sortase tag, an 6xHis tag and a strepII tag.
acggtggctgcaccatctgtcttcatcttcccgccatctgatgagcagttgaaatctggaactgcctctgttgtgtgcctgctgaataacttctatcccagagaggccaaagtacagtggaaggtggataacgccctccaatcgggtaactcccaggagagtgtcacagagcaggacagcaaggacagcacctacagcctcagcagcaccctgacgctgagcaaagcagactacgagaaacacaaagtctacgcctgcgaagtcacccatcagggcctgagctcgcccgtcacaaagagcttcaacaggggagagtgtctgcccgagaccggccaccaccaccaccaccacggcgagcagaagctgatcagcgaggaggacctgggctggagccacccccagttcgagaagtag

SEQ ID NO: 8 - protein, 137 aa, Artificial Sequence
  amino acid sequence of human IgG1 kappa light chain constant region with LPETG sortase tag, an 6xHis tag and a strepII tag.
TVAAPSVFIFPPSDEQLKSGTASVVCLLNNFYPREAKVQWKVDNALQSGNSQESVTEQDSKDSTYSLSSTLTLSKADYEKHKVYACEVTHQGLSSPVTKSFNRGECLPETGHHHHHHGEQKLISEEDLGWSHPQFEK

SEQ ID NO: 9 - DNA, 1503 bp, Artificial Sequence
  Complete human IgG1 VH-CH heavy chain coding region for hBU12 with C-terminal LPETG sortase tag, 6xHis tag and a strepII tag
atgggatggagctggatctttcttttcctcctgtcaggaactgcaggtgtccattgtcaggttcagctgcaagagtctggccctgggttggttaagccctcccagaccctcagtctgacttgtactgtgtctgggggttcaatcagcacttctggtatgggtgtaggctggattaggcagcacccagggaagggtctggagtggattggacacatttggtgggatgatgacaagagatataacccagccctgaagagcagagtgacaatctctgtggatacctccaagaaccagtttagcctcaagctgtccagtgtgacagctgcagatactgctgtctactactgtgctagaatggaactttggtcctactattttgactactggggccaaggcacccttgtcacagtctcctcagctagcaccaagggcccatctgtcttccccctggcaccctcctccaagagcacctctgggggcacagctgccctgggctgcctggtcaaggactacttccctgaacctgtgacagtgtcctggaactcaggcgccctgaccagcggcgtgcacaccttcccggctgtcctacagtcctcaggactctactccctcagcagcgtggtgaccgtgccctccagcagcttgggcacccagacctacatctgcaacgtgaatcacaagcccagcaacaccaaggtggacaagaaagttgagcccaaatcttgtgacaaaactcacacatgcccaccgtgcccagcacctgaactcctggggggaccgtcagtcttcctcttccccccaaaacccaaggacaccctcatgatctcccggacccctgaggtcacatgcgtggtggtggacgtgagccacgaagaccctgaggtcaagttcaactggtacgtggacggcgtggaggtgcataatgccaagacaaagccgcgggaggagcagtacaacagcacgtaccgtgtggtcagcgtcctcaccgtcctgcaccaggactggctgaatggcaaggagtacaagtgcaaggtctccaacaaagccctcccagcccccatcgagaaaaccatctccaaagccaaagggcagccccgagaaccacaggtgtacaccctgcccccatcccgggatgagctgaccaagaaccaggtcagcctgacctgcctggtcaaaggcttctatcccagcgacatcgccgtggagtgggagagcaatgggcagccggagaacaactacaagaccacgcctcccgtgctggactccgacggctccttcttcctctacagcaagctcaccgtggacaagagcaggtggcagcaggggaacgtcttctcatgctccgtgatgcatgaggctctgcacaaccactacacacagaagagcctctccctgtctccgggtaaactgcccgagaccggccaccaccaccaccaccacggcgagcagaagctgatcagcgaggaggacctgggctggagccacccccagttcgagaagtag

SEQ ID NO: 10 - protein, 500 aa, Artificial Sequence
  amino acid sequence of complete human IgG1 VH-CH heavy chain region of hBU12 with C-terminal LPETG sortase tag, 6xHis tag and a strepII tag
MGWSWIFLFLLSGTAGVHCQVQLQESGPGLVKPSQTLSLTCTVSGGSISTSGMGVGWIRQHPGKGLEWIGHIWWDDDKRYNPALKSRVTISVDTSKNQFSLKLSSVTAADTAVYYCARMELWSYYFDYWGQGTLVTVSSASTKGPSVFPLAPSSKSTSGGTAALGCLVKDYFPEPVTVSWNSGALTSGVHTFPAVLQSSGLYSLSSVVTVPSSSLGTQTYICNVNHKPSNTKVDKKVEPKSCDKTHTCPPCPAPELLGGPSVFLFPPKPKDTLMISRTPEVTCVVVDVSHEDPEVKFNWYVDGVEVHNAKTKPREEQYNSTYRVVSVLTVLHQDWLNGKEYKCKVSNKALPAPIEKTISKAKGQPREPQVYTLPPSRDELTKNQVSLTCLVKGFYPSDIAVEWESNGQPENNYKTTPPVLDSDGSFFLYSKLTVDKSRWQQGNVFSCSVMHEALHNHYTQKSLSLSPGKLPETGHHHHHHGEQKLISEEDLGWSHPQFEK

SEQ ID NO: 11 - DNA, 792 bp, Artificial Sequence
  Complete human IgG1 VL-CL kappa chain coding region for hBU12 with C-terminal LPETG sortase tag, 6xHis tag and a strepII tag
atgaagttgcctgttaggctgttggtgctgatgttctggattcctgcttccagcagtgaaattgttctcacccagtctccagcaaccctgtctctctctccaggggaaagggctaccctgagctgcagtgccagctcaagtgtaagttacatgcactggtaccagcagaagccagggcaggctcccagactcctgatttatgacacatccaaactggcttctggtattccagcaaggttcagtggcagtgggtctggaacagattttacactcacaatcagcagcctggagccagaggatgttgctgtctattactgttttcaggggagtgtatacccattcacttttggccaagggacaaagttggaaatcaaaagaactgtggctgcaccatctgtcttcatcttcccgccatctgatgagcagttgaaatctggaactgcctctgttgtgtgcctgctgaataacttctatcccagagaggccaaagtacagtggaaggtggataacgccctccaatcgggtaactcccaggagagtgtcacagagcaggacagcaaggacagcacctacagcctcagcagcaccctgacgctgagcaaagcagactacgagaaacacaaagtctacgcctgcgaagtcacccatcagggcctgagctcgcccgtcacaaagagcttcaacaggggagagtgtctgcccgagaccggccaccaccaccaccaccacggcgagcagaagctgatcagcgaggaggacctgggctggagccacccccagttcgagaagtag

SEQ ID NO: 12 - protein, 263 aa, Artificial Sequence
  amino acid sequence of complete human IgG1 VL-CL kappa chain region of hBU12 with C-terminal LPETG sortase tag, 6xHis tag and a strepII tag
MKLPVRLLVLMFWIPASSSEIVLTQSPATLSLSPGERATLSCSASSSVSYMHWYQQKPGQAPRLLIYDTSKLASGIPARFSGSGSGTDFTLTISSLEPEDVAVYYCFQGSVYPFTFGQGTKLEIKRTVAAPSVFIFPPSDEQLKSGTASVVCLLNNFYPREAKVQWKVDNALQSGNSQESVTEQDSKDSTYSLSSTLTLSKADYEKHKVYACEVTHQGLSSPVTKSFNRGECLPETGHHHHHHGEQKLISEEDLGWSHPQFEK

SEQ ID NO: 13 - DNA, 7045 bp, Artificial Sequence
  coding region of human IgG1 VH-CH heavy chain for hBU12 with C-terminal LPETG sortase tag, 6xHis tag and a strepII tag and HindIII and NotI cloning sites
gacggatcgggagatctcccgatcccctatggtcgactctcagtacaatctgctctgatgccgcatagttaagccagtatctgctccctgcttgtgtgttggaggtcgctgagtagtgcgcgagcaaaatttaagctacaacaaggcaaggcttgaccgacaattgcatgaagaatctgcttagggttaggcgttttgcgctgcttcgcgatgtacgggccagatatacgcgttgacattgattattgactagttattaatagtaatcaattacggggtcattagttcatagcccatatatggagttccgcgttacataacttacggtaaatggcccgcctggctgaccgcccaacgacccccgcccattgacgtcaataatgacgtatgttcccatagtaacgccaatagggactttccattgacgtcaatgggtggactatttacggtaaactgcccacttggcagtacatcaagtgtatcatatgccaagtacgccccctattgacgtcaatgacggtaaatggcccgcctggcattatgcccagtacatgaccttatgggactttcctacttggcagtacatctacgtattagtcatcgctattaccatggtgatgcggttttggcagtacatcaatgggcgtggatagcggtttgactcacggggatttccaagtctccaccccattgacgtcaatgggagtttgttttggcaccaaaatcaacgggactttccaaaatgtcgtaacaactccgccccattgacgcaaatgggcggtaggcgtgtacggtgggaggtctatataagcagagctctctggctaactagagaacccactgcttactggcttatcgaaattaatacgactcactatagggagacccaagctggctagcgtttaaacttaagcttccatgggatggagctggatctttcttttcctcctgtcaggaactgcaggtgtccattgtcaggttcagctgcaagagtctggccctgggttggttaagccctcccagaccctcagtctgacttgtactgtgtctgggggttcaatcagcacttctggtatgggtgtaggctggattaggcagcacccagggaagggtctggagtggattggacacatttggtgggatgatgacaagagatataacccagccctgaagagcagagtgacaatctctgtggatacctccaagaaccagtttagcctcaagctgtccagtgtgacagctgcagatactgctgtctactactgtgctagaatggaactttggtcctactattttgactactggggccaaggcacccttgtcacagtctcctcagctagcaccaagggcccatctgtcttccccctggcaccctcctccaagagcacctctgggggcacagctgccctgggctgcctggtcaaggactacttccctgaacctgtgacagtgtcctggaactcaggcgccctgaccagcggcgtgcacaccttcccggctgtcctacagtcctcaggactctactccctcagcagcgtggtgaccgtgccctccagcagcttgggcacccagacctacatctgcaacgtgaatcacaagcccagcaacaccaaggtggacaagaaagttgagcccaaatcttgtgacaaaactcacacatgcccaccgtgcccagcacctgaactcctggggggaccgtcagtcttcctcttccccccaaaacccaaggacaccctcatgatctcccggacccctgaggtcacatgcgtggtggtggacgtgagccacgaagaccctgaggtcaagttcaactggtacgtggacggcgtggaggtgcataatgccaagacaaagccgcgggaggagcagtacaacagcacgtaccgtgtggtcagcgtcctcaccgtcctgcaccaggactggctgaatggcaaggagtacaagtgcaaggtctccaacaaagccctcccagcccccatcgagaaaaccatctccaaagccaaagggcagccccgagaaccacaggtgtacaccctgcccccatcccgggatgagctgaccaagaaccaggtcagcctgacctgcctggtcaaaggcttctatcccagcgacatcgccgtggagtgggagagcaatgggcagccggagaacaactacaagaccacgcctcccgtgctggactccgacggctccttcttcctctacagcaagctcaccgtggacaagagcaggtggcagcaggggaacgtcttctcatgctccgtgatgcatgaggctctgcacaaccactacacacagaagagcctctccctgtctccgggtaaactgcccgagaccggccaccaccaccaccaccacggcgagcagaagctgatcagcgaggaggacctgggctggagccacccccagttcgagaagtaggcggccgctcgagtctagagggcccgtttaaacccgctgatcagcctcgactgtgccttctagttgccagccatctgttgtttgcccctcccccgtgccttccttgaccctggaaggtgccactcccactgtcctttcctaataaaatgaggaaattgcatcgcattgtctgagtaggtgtcattctattctggggggtggggtggggcaggacagcaagggggaggattgggaagacaatagcaggcatgctggggatgcggtgggctctatggcttctgaggcggaaagaaccagctggggctctagggggtatccccacgcgccctgtagcggcgcattaagcgcggcgggtgtggtggttacgcgcagcgtgaccgctacacttgccagcgccctagcgcccgctcctttcgctttcttcccttcctttctcgccacgttcgccggctttccccgtcaagctctaaatcggggcatccctttagggttccgatttagtgctttacggcacctcgaccccaaaaaacttgattagggtgatggttcacgtagtgggccatcgccctgatagacggtttttcgccctttgacgttggagtccacgttctttaatagtggactcttgttccaaactggaacaacactcaaccctatctcggtctattcttttgatttataagggattttggggatttcggcctattggttaaaaaatgagctgatttaacaaaaatttaacgcgaattaattctgtggaatgtgtgtcagttagggtgtggaaagtccccaggctccccaggcaggcagaagtatgcaaagcatgcatctcaattagtcagcaaccaggtgtggaaagtccccaggctccccagcaggcagaagtatgcaaagcatgcatctcaattagtcagcaaccatagtcccgcccctaactccgcccatcccgcccctaactccgcccagttccgcccattctccgccccatggctgactaattttttttatttatgcagaggccgaggccgcctctgcctctgagctattccagaagtagtgaggaggcttttttggaggcctaggcttttgcaaaaagctcccgggagcttgtatatccattttcggatctgatcagcacgtgatgaaaaagcctgaactcaccgcgacgtctgtcgagaagtttctgatcgaaaagttcgacagcgtctccgacctgatgcagctctcggagggcgaagaatctcgtgctttcagcttcgatgtaggagggcgtggatatgtcctgcgggtaaatagctgcgccgatggtttctacaaagatcgttatgtttatcggcactttgcatcggccgcgctcccgattccggaagtgcttgacattggggaattcagcgagagcctgacctattgcatctcccgccgtgcacagggtgtcacgttgcaagacctgcctgaaaccgaactgcccgctgttctgcagccggtcgcggaggccatggatgcgatcgctgcggccgatcttagccagacgagcgggttcggcccattcggaccgcaaggaatcggtcaatacactacatggcgtgatttcatatgcgcgattgctgatccccatgtgtatcactggcaaactgtgatggacgacaccgtcagtgcgtccgtcgcgcaggctctcgatgagctgatgctttgggccgaggactgccccgaagtccggcacctcgtgcacgcggatttcggctccaacaatgtcctgacggacaatggccgcataacagcggtcattgactggagcgaggcgatgttcggggattcccaatacgaggtcgccaacatcttcttctggaggccgtggttggcttgtatggagcagcagacgcgctacttcgagcggaggcatccggagcttgcaggatcgccgcggctccgggcgtatatgctccgcattggtcttgaccaactctatcagagcttggttgacggcaatttcgatgatgcagcttgggcgcagggtcgatgcgacgcaatcgtccgatccggagccgggactgtcgggcgtacacaaatcgcccgcagaagcgcggccgtctggaccgatggctgtgtagaagtactcgccgatagtggaaaccgacgccccagcactcgtccgagggcaaaggaatagcacgtgctacgagatttcgattccaccgccgccttctatgaaaggttgggcttcggaatcgttttccgggacgccggctggatgatcctccagcgcggggatctcatgctggagttcttcgcccaccccaacttgtttattgcagcttataatggttacaaataaagcaatagcatcacaaatttcacaaataaagcatttttttcactgcattctagttgtggtttgtccaaactcatcaatgtatcttatcatgtctgtataccgtcgacctctagctagagcttggcgtaatcatggtcatagctgtttcctgtgtgaaattgttatccgctcacaattccacacaacatacgagccggaagcataaagtgtaaagcctggggtgcctaatgagtgagctaactcacattaattgcgttgcgctcactgcccgctttccagtcgggaaacctgtcgtgccagctgcattaatgaatcggccaacgcgcggggagaggcggtttgcgtattgggcgctcttccgcttcctcgctcactgactcgctgcgctcggtcgttcggctgcggcgagcggtatcagctcactcaaaggcggtaatacggttatccacagaatcaggggataacgcaggaaagaacatgtgagcaaaaggccagcaaaaggccaggaaccgtaaaaaggccgcgttgctggcgtttttccataggctccgcccccctgacgagcatcacaaaaatcgacgctcaagtcagaggtggcgaaacccgacaggactataaagataccaggcgtttccccctggaagctccctcgtgcgctctcctgttccgaccctgccgcttaccggatacctgtccgcctttctcccttcgggaagcgtggcgctttctcaatgctcacgctgtaggtatctcagttcggtgtaggtcgttcgctccaagctgggctgtgtgcacgaaccccccgttcagcccgaccgctgcgccttatccggtaactatcgtcttgagtccaacccggtaagacacgacttatcgccactggcagcagccactggtaacaggattagcagagcgaggtatgtaggcggtgctacagagttcttgaagtggtggcctaactacggctacactagaaggacagtatttggtatctgcgctctgctgaagccagttaccttcggaaaaagagttggtagctcttgatccggcaaacaaaccaccgctggtagcggtggtttttttgtttgcaagcagcagattacgcgcagaaaaaaaggatctcaagaagatcctttgatcttttctacggggtctgacgctcagtggaacgaaaactcacgttaagggattttggtcatgagattatcaaaaaggatcttcacctagatccttttaaattaaaaatgaagttttaaatcaatctaaagtatatatgagtaaacttggtctgacagttaccaatgcttaatcagtgaggcacctatctcagcgatctgtctatttcgttcatccatagttgcctgactccccgtcgtgtagataactacgatacgggagggcttaccatctggccccagtgctgcaatgataccgcgagacccacgctcaccggctccagatttatcagcaataaaccagccagccggaagggccgagcgcagaagtggtcctgcaactttatccgcctccatccagtctattaattgttgccgggaagctagagtaagtagttcgccagttaatagtttgcgcaacgttgttgccattgctacaggcatcgtggtgtcacgctcgtcgtttggtatggcttcattcagctccggttcccaacgatcaaggcgagttacatgatcccccatgttgtgcaaaaaagcggttagctccttcggtcctccgatcgttgtcagaagtaagttggccgcagtgttatcactcatggttatggcagcactgcataattctcttactgtcatgccatccgtaagatgcttttctgtgactggtgagtactcaaccaagtcattctgagaatagtgtatgcggcgaccgagttgctcttgcccggcgtcaatacgggataataccgcgccacatagcagaactttaaaagtgctcatcattggaaaacgttcttcggggcgaaaactctcaaggatcttaccgctgttgagatccagttcgatgtaacccactcgtgcacccaactgatcttcagcatcttttactttcaccagcgtttctgggtgagcaaaaacaggaaggcaaaatgccgcaaaaaagggaataagggcgacacggaaatgttgaatactcatactcttcctttttcaatattattgaagcatttatcagggttattgtctcatgagcggatacatatttgaatgtatttagaaaaataaacaaataggggttccgcgcacatttccccgaaaagtgccacctgacgtc

SEQ ID NO: 14 - DNA, 6334 bp, Artificial Sequence
  coding region of human IgG1 VL-CL kappa light chain for hBU12 with C-terminal LPETG sortase tag, 6xHis tag and a strepII tag and HindIII and NotI cloning sites
gacggatcgggagatctcccgatcccctatggtcgactctcagtacaatctgctctgatgccgcatagttaagccagtatctgctccctgcttgtgtgttggaggtcgctgagtagtgcgcgagcaaaatttaagctacaacaaggcaaggcttgaccgacaattgcatgaagaatctgcttagggttaggcgttttgcgctgcttcgcgatgtacgggccagatatacgcgttgacattgattattgactagttattaatagtaatcaattacggggtcattagttcatagcccatatatggagttccgcgttacataacttacggtaaatggcccgcctggctgaccgcccaacgacccccgcccattgacgtcaataatgacgtatgttcccatagtaacgccaatagggactttccattgacgtcaatgggtggactatttacggtaaactgcccacttggcagtacatcaagtgtatcatatgccaagtacgccccctattgacgtcaatgacggtaaatggcccgcctggcattatgcccagtacatgaccttatgggactttcctacttggcagtacatctacgtattagtcatcgctattaccatggtgatgcggttttggcagtacatcaatgggcgtggatagcggtttgactcacggggatttccaagtctccaccccattgacgtcaatgggagtttgttttggcaccaaaatcaacgggactttccaaaatgtcgtaacaactccgccccattgacgcaaatgggcggtaggcgtgtacggtgggaggtctatataagcagagctctctggctaactagagaacccactgcttactggcttatcgaaattaatacgactcactatagggagacccaagctggctagcgtttaaacttaagcttccatgaagttgcctgttaggctgttggtgctgatgttctggattcctgcttccagcagtgaaattgttctcacccagtctccagcaaccctgtctctctctccaggggaaagggctaccctgagctgcagtgccagctcaagtgtaagttacatgcactggtaccagcagaagccagggcaggctcccagactcctgatttatgacacatccaaactggcttctggtattccagcaaggttcagtggcagtgggtctggaacagattttacactcacaatcagcagcctggagccagaggatgttgctgtctattactgttttcaggggagtgtatacccattcacttttggccaagggacaaagttggaaatcaaaagaactgtggctgcaccatctgtcttcatcttcccgccatctgatgagcagttgaaatctggaactgcctctgttgtgtgcctgctgaataacttctatcccagagaggccaaagtacagtggaaggtggataacgccctccaatcgggtaactcccaggagagtgtcacagagcaggacagcaaggacagcacctacagcctcagcagcaccctgacgctgagcaaagcagactacgagaaacacaaagtctacgcctgcgaagtcacccatcagggcctgagctcgcccgtcacaaagagcttcaacaggggagagtgtctgcccgagaccggccaccaccaccaccaccacggcgagcagaagctgatcagcgaggaggacctgggctggagccacccccagttcgagaagtaggcggccgctcgagtctagagggcccgtttaaacccgctgatcagcctcgactgtgccttctagttgccagccatctgttgtttgcccctcccccgtgccttccttgaccctggaaggtgccactcccactgtcctttcctaataaaatgaggaaattgcatcgcattgtctgagtaggtgtcattctattctggggggtggggtggggcaggacagcaagggggaggattgggaagacaatagcaggcatgctggggatgcggtgggctctatggcttctgaggcggaaagaaccagctggggctctagggggtatccccacgcgccctgtagcggcgcattaagcgcggcgggtgtggtggttacgcgcagcgtgaccgctacacttgccagcgccctagcgcccgctcctttcgctttcttcccttcctttctcgccacgttcgccggctttccccgtcaagctctaaatcggggcatccctttagggttccgatttagtgctttacggcacctcgaccccaaaaaacttgattagggtgatggttcacgtagtgggccatcgccctgatagacggtttttcgccctttgacgttggagtccacgttctttaatagtggactcttgttccaaactggaacaacactcaaccctatctcggtctattcttttgatttataagggattttggggatttcggcctattggttaaaaaatgagctgatttaacaaaaatttaacgcgaattaattctgtggaatgtgtgtcagttagggtgtggaaagtccccaggctccccaggcaggcagaagtatgcaaagcatgcatctcaattagtcagcaaccaggtgtggaaagtccccaggctccccagcaggcagaagtatgcaaagcatgcatctcaattagtcagcaaccatagtcccgcccctaactccgcccatcccgcccctaactccgcccagttccgcccattctccgccccatggctgactaattttttttatttatgcagaggccgaggccgcctctgcctctgagctattccagaagtagtgaggaggcttttttggaggcctaggcttttgcaaaaagctcccgggagcttgtatatccattttcggatctgatcagcacgtgatgaaaaagcctgaactcaccgcgacgtctgtcgagaagtttctgatcgaaaagttcgacagcgtctccgacctgatgcagctctcggagggcgaagaatctcgtgctttcagcttcgatgtaggagggcgtggatatgtcctgcgggtaaatagctgcgccgatggtttctacaaagatcgttatgtttatcggcactttgcatcggccgcgctcccgattccggaagtgcttgacattggggaattcagcgagagcctgacctattgcatctcccgccgtgcacagggtgtcacgttgcaagacctgcctgaaaccgaactgcccgctgttctgcagccggtcgcggaggccatggatgcgatcgctgcggccgatcttagccagacgagcgggttcggcccattcggaccgcaaggaatcggtcaatacactacatggcgtgatttcatatgcgcgattgctgatccccatgtgtatcactggcaaactgtgatggacgacaccgtcagtgcgtccgtcgcgcaggctctcgatgagctgatgctttgggccgaggactgccccgaagtccggcacctcgtgcacgcggatttcggctccaacaatgtcctgacggacaatggccgcataacagcggtcattgactggagcgaggcgatgttcggggattcccaatacgaggtcgccaacatcttcttctggaggccgtggttggcttgtatggagcagcagacgcgctacttcgagcggaggcatccggagcttgcaggatcgccgcggctccgggcgtatatgctccgcattggtcttgaccaactctatcagagcttggttgacggcaatttcgatgatgcagcttgggcgcagggtcgatgcgacgcaatcgtccgatccggagccgggactgtcgggcgtacacaaatcgcccgcagaagcgcggccgtctggaccgatggctgtgtagaagtactcgccgatagtggaaaccgacgccccagcactcgtccgagggcaaaggaatagcacgtgctacgagatttcgattccaccgccgccttctatgaaaggttgggcttcggaatcgttttccgggacgccggctggatgatcctccagcgcggggatctcatgctggagttcttcgcccaccccaacttgtttattgcagcttataatggttacaaataaagcaatagcatcacaaatttcacaaataaagcatttttttcactgcattctagttgtggtttgtccaaactcatcaatgtatcttatcatgtctgtataccgtcgacctctagctagagcttggcgtaatcatggtcatagctgtttcctgtgtgaaattgttatccgctcacaattccacacaacatacgagccggaagcataaagtgtaaagcctggggtgcctaatgagtgagctaactcacattaattgcgttgcgctcactgcccgctttccagtcgggaaacctgtcgtgccagctgcattaatgaatcggccaacgcgcggggagaggcggtttgcgtattgggcgctcttccgcttcctcgctcactgactcgctgcgctcggtcgttcggctgcggcgagcggtatcagctcactcaaaggcggtaatacggttatccacagaatcaggggataacgcaggaaagaacatgtgagcaaaaggccagcaaaaggccaggaaccgtaaaaaggccgcgttgctggcgtttttccataggctccgcccccctgacgagcatcacaaaaatcgacgctcaagtcagaggtggcgaaacccgacaggactataaagataccaggcgtttccccctggaagctccctcgtgcgctctcctgttccgaccctgccgcttaccggatacctgtccgcctttctcccttcgggaagcgtggcgctttctcaatgctcacgctgtaggtatctcagttcggtgtaggtcgttcgctccaagctgggctgtgtgcacgaaccccccgttcagcccgaccgctgcgccttatccggtaactatcgtcttgagtccaacccggtaagacacgacttatcgccactggcagcagccactggtaacaggattagcagagcgaggtatgtaggcggtgctacagagttcttgaagtggtggcctaactacggctacactagaaggacagtatttggtatctgcgctctgctgaagccagttaccttcggaaaaagagttggtagctcttgatccggcaaacaaaccaccgctggtagcggtggtttttttgtttgcaagcagcagattacgcgcagaaaaaaaggatctcaagaagatcctttgatcttttctacggggtctgacgctcagtggaacgaaaactcacgttaagggattttggtcatgagattatcaaaaaggatcttcacctagatccttttaaattaaaaatgaagttttaaatcaatctaaagtatatatgagtaaacttggtctgacagttaccaatgcttaatcagtgaggcacctatctcagcgatctgtctatttcgttcatccatagttgcctgactccccgtcgtgtagataactacgatacgggagggcttaccatctggccccagtgctgcaatgataccgcgagacccacgctcaccggctccagatttatcagcaataaaccagccagccggaagggccgagcgcagaagtggtcctgcaactttatccgcctccatccagtctattaattgttgccgggaagctagagtaagtagttcgccagttaatagtttgcgcaacgttgttgccattgctacaggcatcgtggtgtcacgctcgtcgtttggtatggcttcattcagctccggttcccaacgatcaaggcgagttacatgatcccccatgttgtgcaaaaaagcggttagctccttcggtcctccgatcgttgtcagaagtaagttggccgcagtgttatcactcatggttatggcagcactgcataattctcttactgtcatgccatccgtaagatgcttttctgtgactggtgagtactcaaccaagtcattctgagaatagtgtatgcggcgaccgagttgctcttgcccggcgtcaatacgggataataccgcgccacatagcagaactttaaaagtgctcatcattggaaaacgttcttcggggcgaaaactctcaaggatcttaccgctgttgagatccagttcgatgtaacccactcgtgcacccaactgatcttcagcatcttttactttcaccagcgtttctgggtgagcaaaaacaggaaggcaaaatgccgcaaaaaagggaataagggcgacacggaaatgttgaatactcatactcttcctttttcaatattattgaagcatttatcagggttattgtctcatgagcggatacatatttgaatgtatttagaaaaataaacaaataggggttccgcgcacatttccccgaaaagtgccacctgacgtc

SEQ ID NO: 15 - protein, 150 aa, Artificial Sequence
  amino acid sequence of the N-intein domain of Ssp GyrB 11 split-intein
CFSGDTLVALTDGRSVSFEQLVEEEKQGKQNFCYTIRHDGSIGVEKIINARKTKTNAKVIKVTLDNGESIICTPDHKFMLRDGSYKCAMDLTLDDSLMPLHRKISTTEDSGHMEAVLNYNHRIVNIEAVSETIDVYDIEVPHTHNFALAS

SEQ ID NO: 16 - DNA, 450 bp, Artificial Sequence
  Reverse translation of SEQ ID NO 15 with mammalian codon usage results in the coding sequence for the N-intein domain of Ssp GyrB 11 split-intein
tgcttcagcggcgacaccctggtggccctgaccgacggcagaagcgtgagcttcgagcagctggtggaggaggagaagcagggcaagcagaacttctgctacaccatcagacacgacggcagcatcggcgtggagaagatcatcaacgccagaaagaccaagaccaacgccaaggtgatcaaggtgaccctggacaacggcgagagcatcatctgcacccccgaccacaagttcatgctgagagacggcagctacaagtgcgccatggacctgaccctggacgacagcctgatgcccctgcacagaaagatcagcaccaccgaggacagcggccacatggaggccgtgctgaactacaaccacagaatcgtgaacatcgaggccgtgagcgagaccatcgacgtgtacgacatcgaggtgccccacacccacaacttcgccctggccagc

SEQ ID NO: 17 - DNA, 1905 bp, Artificial Sequence
  complete IgG1 heavy chain coding region for anti-human CD19 antibody hBU12 with C-terminal extension, comprising the N-intein domain of Ssp GyrB 11 split-intein, followed by a 6xHis-tag and a strepII tag
atgaattttggactgaggctgattttcctggtgctgaccctgaaaggcgtccagtgtcaggttcagctgcaagagtctggccctgggttggttaagccctcccagaccctcagtctgacttgtactgtgtctgggggttcaatcagcacttctggtatgggtgtaggctggattaggcagcacccagggaagggtctggagtggattggacacatttggtgggatgatgacaagagatataacccagccctgaagagcagagtgacaatctctgtggatacctccaagaaccagtttagcctcaagctgtccagtgtgacagctgcagatactgctgtctactactgtgctagaatggaactttggtcctactattttgactactggggccaaggcacccttgtcacagtctcctcagctagcaccaagggcccatctgtcttccccctggcaccctcctccaagagcacctctgggggcacagctgccctgggctgcctggtcaaggactacttccctgaacctgtgacagtgtcctggaactcaggcgccctgaccagcggcgtgcacaccttcccggctgtcctacagtcctcaggactctactccctcagcagcgtggtgaccgtgccctccagcagcttgggcacccagacctacatctgcaacgtgaatcacaagcccagcaacaccaaggtggacaagaaagttgagcccaaatcttgtgacaaaactcacacatgcccaccgtgcccagcacctgaactcctggggggaccgtcagtcttcctcttccccccaaaacccaaggacaccctcatgatctcccggacccctgaggtcacatgcgtggtggtggacgtgagccacgaagaccctgaggtcaagttcaactggtacgtggacggcgtggaggtgcataatgccaagacaaagccgcgggaggagcagtacaacagcacgtaccgtgtggtcagcgtcctcaccgtcctgcaccaggactggctgaatggcaaggagtacaagtgcaaggtctccaacaaagccctcccagcccccatcgagaaaaccatctccaaagccaaagggcagccccgagaaccacaggtgtacaccctgcccccatcccgggatgagctgaccaagaaccaggtcagcctgacctgcctggtcaaaggcttctatcccagcgacatcgccgtggagtgggagagcaatgggcagccggagaacaactacaagaccacgcctcccgtgctggactccgacggctccttcttcctctacagcaagctcaccgtggacaagagcaggtggcagcaggggaacgtcttctcatgctccgtgatgcatgaggctctgcacaaccactacacacagaagagcctctccctgtctccgggtaaatgcttcagcggcgacaccctggtggccctgaccgacggcagaagcgtgagcttcgagcagctggtggaggaggagaagcagggcaagcagaacttctgctacaccatcagacacgacggcagcatcggcgtggagaagatcatcaacgccagaaagaccaagaccaacgccaaggtgatcaaggtgaccctggacaacggcgagagcatcatctgcacccccgaccacaagttcatgctgagagacggcagctacaagtgcgccatggacctgaccctggacgacagcctgatgcccctgcacagaaagatcagcaccaccgaggacagcggccacatggaggccgtgctgaactacaaccacagaatcgtgaacatcgaggccgtgagcgagaccatcgacgtgtacgacatcgaggtgccccacacccacaacttcgccctggccagccaccatcaccatcaccatggctggagccacccccagttcgagaagtag

SEQ ID NO: 18 - protein, 634 aa, Artificial Sequence
  Amino acid sequence translated from SEQ ID NO 17
MNFGLRLIFLVLTLKGVQCQVQLQESGPGLVKPSQTLSLTCTVSGGSISTSGMGVGWIRQHPGKGLEWIGHIWWDDDKRYNPALKSRVTISVDTSKNQFSLKLSSVTAADTAVYYCARMELWSYYFDYWGQGTLVTVSSASTKGPSVFPLAPSSKSTSGGTAALGCLVKDYFPEPVTVSWNSGALTSGVHTFPAVLQSSGLYSLSSVVTVPSSSLGTQTYICNVNHKPSNTKVDKKVEPKSCDKTHTCPPCPAPELLGGPSVFLFPPKPKDTLMISRTPEVTCVVVDVSHEDPEVKFNWYVDGVEVHNAKTKPREEQYNSTYRVVSVLTVLHQDWLNGKEYKCKVSNKALPAPIEKTISKAKGQPREPQVYTLPPSRDELTKNQVSLTCLVKGFYPSDIAVEWESNGQPENNYKTTPPVLDSDGSFFLYSKLTVDKSRWQQGNVFSCSVMHEALHNHYTQKSLSLSPGKCFSGDTLVALTDGRSVSFEQLVEEEKQGKQNFCYTIRHDGSIGVEKIINARKTKTNAKVIKVTLDNGESIICTPDHKFMLRDGSYKCAMDLTLDDSLMPLHRKISTTEDSGHMEAVLNYNHRIVNIEAVSETIDVYDIEVPHTHNFALASHHHHHHGWSHPQFEK

SEQ ID NO: 19 - DNA, 1206 bp, Artificial Sequence
  complete IgG1 kappa light chain coding region for anti-human CD19 antibody hBU12 with C-terminal extension, comprising the N-intein domain of Ssp GyrB 11 split-intein, followed by a 6xHis-tag and a strepII tag
atgaattttggactgaggctgattttcctggtgctgaccctgaaaggcgtccagtgtgacattgtgctgacccaatctccagcttctttggctgtgtctctagggcagagggccaccatctcctgcaaggccagccaaagtgttgattttgatggtgatagttatatgaactggtaccaacagaaaccaggacagccacccaaagtcctcatctatgctgcatccaatctagaatctgggatcccagccaggtttagtggcagtgggtctgggacagacttcaccctcaacatccatcctgtggaggaggaggatgctgcaacctattactgtcagcaaagtaatgaggatccgtggacgttcggtggaggcaccaagctggaaatcaaacgtacggtggctgcaccatctgtcttcatcttcccgccatctgatgagcagttgaaatctggaactgcctctgttgtgtgcctgctgaataacttctatcccagagaggccaaagtacagtggaaggtggataacgccctccaatcgggtaactcccaggagagtgtcacagagcaggacagcaaggacagcacctacagcctcagcagcaccctgacgctgagcaaagcagactacgagaaacacaaagtctacgcctgcgaagtcacccatcagggcctgagctcgcccgtcacaaagagcttcaacaggggagagtgcttcagcggcgacaccctggtggccctgaccgacggcagaagcgtgagcttcgagcagctggtggaggaggagaagcagggcaagcagaacttctgctacaccatcagacacgacggcagcatcggcgtggagaagatcatcaacgccagaaagaccaagaccaacgccaaggtgatcaaggtgaccctggacaacggcgagagcatcatctgcacccccgaccacaagttcatgctgagagacggcagctacaagtgcgccatggacctgaccctggacgacagcctgatgcccctgcacagaaagatcagcaccaccgaggacagcggccacatggaggccgtgctgaactacaaccacagaatcgtgaacatcgaggccgtgagcgagaccatcgacgtgtacgacatcgaggtgccccacacccacaacttcgccctggccagccaccatcaccatcaccatggctggagccacccccagttcgagaagtag

SEQ ID NO: 20 - protein, 401 aa, Artificial Sequence
  Amino acid sequence translated from SEQ ID NO 19
MNFGLRLIFLVLTLKGVQCDIVLTQSPASLAVSLGQRATISCKASQSVDFDGDSYMNWYQQKPGQPPKVLIYAASNLESGIPARFSGSGSGTDFTLNIHPVEEEDAATYYCQQSNEDPWTFGGGTKLEIKRTVAAPSVFIFPPSDEQLKSGTASVVCLLNNFYPREAKVQWKVDNALQSGNSQESVTEQDSKDSTYSLSSTLTLSKADYEKHKVYACEVTHQGLSSPVTKSFNRGECFSGDTLVALTDGRSVSFEQLVEEEKQGKQNFCYTIRHDGSIGVEKIINARKTKTNAKVIKVTLDNGESIICTPDHKFMLRDGSYKCAMDLTLDDSLMPLHRKISTTEDSGHMEAVLNYNHRIVNIEAVSETIDVYDIEVPHTHNFALASHHHHHHGWSHPQFEK

SEQ ID NO: 21 - DNA, 7447 bp, Artificial Sequence
  coding region of human IgG1 VH-CH heavy chain for hBU12 with C-terminal N-intein domain of Ssp GyrB S11 split intein, followed by 6xHis tag strepII tag and HindIII and NotI cloning sites
gacggatcgggagatctcccgatcccctatggtcgactctcagtacaatctgctctgatgccgcatagttaagccagtatctgctccctgcttgtgtgttggaggtcgctgagtagtgcgcgagcaaaatttaagctacaacaaggcaaggcttgaccgacaattgcatgaagaatctgcttagggttaggcgttttgcgctgcttcgcgatgtacgggccagatatacgcgttgacattgattattgactagttattaatagtaatcaattacggggtcattagttcatagcccatatatggagttccgcgttacataacttacggtaaatggcccgcctggctgaccgcccaacgacccccgcccattgacgtcaataatgacgtatgttcccatagtaacgccaatagggactttccattgacgtcaatgggtggactatttacggtaaactgcccacttggcagtacatcaagtgtatcatatgccaagtacgccccctattgacgtcaatgacggtaaatggcccgcctggcattatgcccagtacatgaccttatgggactttcctacttggcagtacatctacgtattagtcatcgctattaccatggtgatgcggttttggcagtacatcaatgggcgtggatagcggtttgactcacggggatttccaagtctccaccccattgacgtcaatgggagtttgttttggcaccaaaatcaacgggactttccaaaatgtcgtaacaactccgccccattgacgcaaatgggcggtaggcgtgtacggtgggaggtctatataagcagagctctctggctaactagagaacccactgcttactggcttatcgaaattaatacgactcactatagggagacccaagctggctagcgtttaaacttaagcttccatgaattttggactgaggctgattttcctggtgctgaccctgaaaggcgtccagtgtcaggttcagctgcaagagtctggccctgggttggttaagccctcccagaccctcagtctgacttgtactgtgtctgggggttcaatcagcacttctggtatgggtgtaggctggattaggcagcacccagggaagggtctggagtggattggacacatttggtgggatgatgacaagagatataacccagccctgaagagcagagtgacaatctctgtggatacctccaagaaccagtttagcctcaagctgtccagtgtgacagctgcagatactgctgtctactactgtgctagaatggaactttggtcctactattttgactactggggccaaggcacccttgtcacagtctcctcagctagcaccaagggcccatctgtcttccccctggcaccctcctccaagagcacctctgggggcacagctgccctgggctgcctggtcaaggactacttccctgaacctgtgacagtgtcctggaactcaggcgccctgaccagcggcgtgcacaccttcccggctgtcctacagtcctcaggactctactccctcagcagcgtggtgaccgtgccctccagcagcttgggcacccagacctacatctgcaacgtgaatcacaagcccagcaacaccaaggtggacaagaaagttgagcccaaatcttgtgacaaaactcacacatgcccaccgtgcccagcacctgaactcctggggggaccgtcagtcttcctcttccccccaaaacccaaggacaccctcatgatctcccggacccctgaggtcacatgcgtggtggtggacgtgagccacgaagaccctgaggtcaagttcaactggtacgtggacggcgtggaggtgcataatgccaagacaaagccgcgggaggagcagtacaacagcacgtaccgtgtggtcagcgtcctcaccgtcctgcaccaggactggctgaatggcaaggagtacaagtgcaaggtctccaacaaagccctcccagcccccatcgagaaaaccatctccaaagccaaagggcagccccgagaaccacaggtgtacaccctgcccccatcccgggatgagctgaccaagaaccaggtcagcctgacctgcctggtcaaaggcttctatcccagcgacatcgccgtggagtgggagagcaatgggcagccggagaacaactacaagaccacgcctcccgtgctggactccgacggctccttcttcctctacagcaagctcaccgtggacaagagcaggtggcagcaggggaacgtcttctcatgctccgtgatgcatgaggctctgcacaaccactacacacagaagagcctctccctgtctccgggtaaatgcttcagcggcgacaccctggtggccctgaccgacggcagaagcgtgagcttcgagcagctggtggaggaggagaagcagggcaagcagaacttctgctacaccatcagacacgacggcagcatcggcgtggagaagatcatcaacgccagaaagaccaagaccaacgccaaggtgatcaaggtgaccctggacaacggcgagagcatcatctgcacccccgaccacaagttcatgctgagagacggcagctacaagtgcgccatggacctgaccctggacgacagcctgatgcccctgcacagaaagatcagcaccaccgaggacagcggccacatggaggccgtgctgaactacaaccacagaatcgtgaacatcgaggccgtgagcgagaccatcgacgtgtacgacatcgaggtgccccacacccacaacttcgccctggccagccaccatcaccatcaccatggctggagccacccccagttcgagaagtaggcggccgctcgagtctagagggcccgtttaaacccgctgatcagcctcgactgtgccttctagttgccagccatctgttgtttgcccctcccccgtgccttccttgaccctggaaggtgccactcccactgtcctttcctaataaaatgaggaaattgcatcgcattgtctgagtaggtgtcattctattctggggggtggggtggggcaggacagcaagggggaggattgggaagacaatagcaggcatgctggggatgcggtgggctctatggcttctgaggcggaaagaaccagctggggctctagggggtatccccacgcgccctgtagcggcgcattaagcgcggcgggtgtggtggttacgcgcagcgtgaccgctacacttgccagcgccctagcgcccgctcctttcgctttcttcccttcctttctcgccacgttcgccggctttccccgtcaagctctaaatcggggcatccctttagggttccgatttagtgctttacggcacctcgaccccaaaaaacttgattagggtgatggttcacgtagtgggccatcgccctgatagacggtttttcgccctttgacgttggagtccacgttctttaatagtggactcttgttccaaactggaacaacactcaaccctatctcggtctattcttttgatttataagggattttggggatttcggcctattggttaaaaaatgagctgatttaacaaaaatttaacgcgaattaattctgtggaatgtgtgtcagttagggtgtggaaagtccccaggctccccaggcaggcagaagtatgcaaagcatgcatctcaattagtcagcaaccaggtgtggaaagtccccaggctccccagcaggcagaagtatgcaaagcatgcatctcaattagtcagcaaccatagtcccgcccctaactccgcccatcccgcccctaactccgcccagttccgcccattctccgccccatggctgactaattttttttatttatgcagaggccgaggccgcctctgcctctgagctattccagaagtagtgaggaggcttttttggaggcctaggcttttgcaaaaagctcccgggagcttgtatatccattttcggatctgatcagcacgtgatgaaaaagcctgaactcaccgcgacgtctgtcgagaagtttctgatcgaaaagttcgacagcgtctccgacctgatgcagctctcggagggcgaagaatctcgtgctttcagcttcgatgtaggagggcgtggatatgtcctgcgggtaaatagctgcgccgatggtttctacaaagatcgttatgtttatcggcactttgcatcggccgcgctcccgattccggaagtgcttgacattggggaattcagcgagagcctgacctattgcatctcccgccgtgcacagggtgtcacgttgcaagacctgcctgaaaccgaactgcccgctgttctgcagccggtcgcggaggccatggatgcgatcgctgcggccgatcttagccagacgagcgggttcggcccattcggaccgcaaggaatcggtcaatacactacatggcgtgatttcatatgcgcgattgctgatccccatgtgtatcactggcaaactgtgatggacgacaccgtcagtgcgtccgtcgcgcaggctctcgatgagctgatgctttgggccgaggactgccccgaagtccggcacctcgtgcacgcggatttcggctccaacaatgtcctgacggacaatggccgcataacagcggtcattgactggagcgaggcgatgttcggggattcccaatacgaggtcgccaacatcttcttctggaggccgtggttggcttgtatggagcagcagacgcgctacttcgagcggaggcatccggagcttgcaggatcgccgcggctccgggcgtatatgctccgcattggtcttgaccaactctatcagagcttggttgacggcaatttcgatgatgcagcttgggcgcagggtcgatgcgacgcaatcgtccgatccggagccgggactgtcgggcgtacacaaatcgcccgcagaagcgcggccgtctggaccgatggctgtgtagaagtactcgccgatagtggaaaccgacgccccagcactcgtccgagggcaaaggaatagcacgtgctacgagatttcgattccaccgccgccttctatgaaaggttgggcttcggaatcgttttccgggacgccggctggatgatcctccagcgcggggatctcatgctggagttcttcgcccaccccaacttgtttattgcagcttataatggttacaaataaagcaatagcatcacaaatttcacaaataaagcatttttttcactgcattctagttgtggtttgtccaaactcatcaatgtatcttatcatgtctgtataccgtcgacctctagctagagcttggcgtaatcatggtcatagctgtttcctgtgtgaaattgttatccgctcacaattccacacaacatacgagccggaagcataaagtgtaaagcctggggtgcctaatgagtgagctaactcacattaattgcgttgcgctcactgcccgctttccagtcgggaaacctgtcgtgccagctgcattaatgaatcggccaacgcgcggggagaggcggtttgcgtattgggcgctcttccgcttcctcgctcactgactcgctgcgctcggtcgttcggctgcggcgagcggtatcagctcactcaaaggcggtaatacggttatccacagaatcaggggataacgcaggaaagaacatgtgagcaaaaggccagcaaaaggccaggaaccgtaaaaaggccgcgttgctggcgtttttccataggctccgcccccctgacgagcatcacaaaaatcgacgctcaagtcagaggtggcgaaacccgacaggactataaagataccaggcgtttccccctggaagctccctcgtgcgctctcctgttccgaccctgccgcttaccggatacctgtccgcctttctcccttcgggaagcgtggcgctttctcaatgctcacgctgtaggtatctcagttcggtgtaggtcgttcgctccaagctgggctgtgtgcacgaaccccccgttcagcccgaccgctgcgccttatccggtaactatcgtcttgagtccaacccggtaagacacgacttatcgccactggcagcagccactggtaacaggattagcagagcgaggtatgtaggcggtgctacagagttcttgaagtggtggcctaactacggctacactagaaggacagtatttggtatctgcgctctgctgaagccagttaccttcggaaaaagagttggtagctcttgatccggcaaacaaaccaccgctggtagcggtggtttttttgtttgcaagcagcagattacgcgcagaaaaaaaggatctcaagaagatcctttgatcttttctacggggtctgacgctcagtggaacgaaaactcacgttaagggattttggtcatgagattatcaaaaaggatcttcacctagatccttttaaattaaaaatgaagttttaaatcaatctaaagtatatatgagtaaacttggtctgacagttaccaatgcttaatcagtgaggcacctatctcagcgatctgtctatttcgttcatccatagttgcctgactccccgtcgtgtagataactacgatacgggagggcttaccatctggccccagtgctgcaatgataccgcgagacccacgctcaccggctccagatttatcagcaataaaccagccagccggaagggccgagcgcagaagtggtcctgcaactttatccgcctccatccagtctattaattgttgccgggaagctagagtaagtagttcgccagttaatagtttgcgcaacgttgttgccattgctacaggcatcgtggtgtcacgctcgtcgtttggtatggcttcattcagctccggttcccaacgatcaaggcgagttacatgatcccccatgttgtgcaaaaaagcggttagctccttcggtcctccgatcgttgtcagaagtaagttggccgcagtgttatcactcatggttatggcagcactgcataattctcttactgtcatgccatccgtaagatgcttttctgtgactggtgagtactcaaccaagtcattctgagaatagtgtatgcggcgaccgagttgctcttgcccggcgtcaatacgggataataccgcgccacatagcagaactttaaaagtgctcatcattggaaaacgttcttcggggcgaaaactctcaaggatcttaccgctgttgagatccagttcgatgtaacccactcgtgcacccaactgatcttcagcatcttttactttcaccagcgtttctgggtgagcaaaaacaggaaggcaaaatgccgcaaaaaagggaataagggcgacacggaaatgttgaatactcatactcttcctttttcaatattattgaagcatttatcagggttattgtctcatgagcggatacatatttgaatgtatttagaaaaataaacaaataggggttccgcgcacatttccccgaaaagtgccacctgacgtc

SEQ ID NO: 22 - DNA, 6748 bp, Artificial Sequence
  coding region of human IgG1 VL-CL kappa light chain for hBU12 with C-terminal Ssp GyrB S11 N-intein domain, 6xHis tag and a strepII tag, and HindIII and NotI cloning sites
gacggatcgggagatctcccgatcccctatggtcgactctcagtacaatctgctctgatgccgcatagttaagccagtatctgctccctgcttgtgtgttggaggtcgctgagtagtgcgcgagcaaaatttaagctacaacaaggcaaggcttgaccgacaattgcatgaagaatctgcttagggttaggcgttttgcgctgcttcgcgatgtacgggccagatatacgcgttgacattgattattgactagttattaatagtaatcaattacggggtcattagttcatagcccatatatggagttccgcgttacataacttacggtaaatggcccgcctggctgaccgcccaacgacccccgcccattgacgtcaataatgacgtatgttcccatagtaacgccaatagggactttccattgacgtcaatgggtggactatttacggtaaactgcccacttggcagtacatcaagtgtatcatatgccaagtacgccccctattgacgtcaatgacggtaaatggcccgcctggcattatgcccagtacatgaccttatgggactttcctacttggcagtacatctacgtattagtcatcgctattaccatggtgatgcggttttggcagtacatcaatgggcgtggatagcggtttgactcacggggatttccaagtctccaccccattgacgtcaatgggagtttgttttggcaccaaaatcaacgggactttccaaaatgtcgtaacaactccgccccattgacgcaaatgggcggtaggcgtgtacggtgggaggtctatataagcagagctctctggctaactagagaacccactgcttactggcttatcgaaattaatacgactcactatagggagacccaagctggctagcgtttaaacttaagcttccatgaattttggactgaggctgattttcctggtgctgaccctgaaaggcgtccagtgtgacattgtgctgacccaatctccagcttctttggctgtgtctctagggcagagggccaccatctcctgcaaggccagccaaagtgttgattttgatggtgatagttatatgaactggtaccaacagaaaccaggacagccacccaaagtcctcatctatgctgcatccaatctagaatctgggatcccagccaggtttagtggcagtgggtctgggacagacttcaccctcaacatccatcctgtggaggaggaggatgctgcaacctattactgtcagcaaagtaatgaggatccgtggacgttcggtggaggcaccaagctggaaatcaaacgtacggtggctgcaccatctgtcttcatcttcccgccatctgatgagcagttgaaatctggaactgcctctgttgtgtgcctgctgaataacttctatcccagagaggccaaagtacagtggaaggtggataacgccctccaatcgggtaactcccaggagagtgtcacagagcaggacagcaaggacagcacctacagcctcagcagcaccctgacgctgagcaaagcagactacgagaaacacaaagtctacgcctgcgaagtcacccatcagggcctgagctcgcccgtcacaaagagcttcaacaggggagagtgcttcagcggcgacaccctggtggccctgaccgacggcagaagcgtgagcttcgagcagctggtggaggaggagaagcagggcaagcagaacttctgctacaccatcagacacgacggcagcatcggcgtggagaagatcatcaacgccagaaagaccaagaccaacgccaaggtgatcaaggtgaccctggacaacggcgagagcatcatctgcacccccgaccacaagttcatgctgagagacggcagctacaagtgcgccatggacctgaccctggacgacagcctgatgcccctgcacagaaagatcagcaccaccgaggacagcggccacatggaggccgtgctgaactacaaccacagaatcgtgaacatcgaggccgtgagcgagaccatcgacgtgtacgacatcgaggtgccccacacccacaacttcgccctggccagccaccatcaccatcaccatggctggagccacccccagttcgagaagtaggcggccgctcgagtctagagggcccgtttaaacccgctgatcagcctcgactgtgccttctagttgccagccatctgttgtttgcccctcccccgtgccttccttgaccctggaaggtgccactcccactgtcctttcctaataaaatgaggaaattgcatcgcattgtctgagtaggtgtcattctattctggggggtggggtggggcaggacagcaagggggaggattgggaagacaatagcaggcatgctggggatgcggtgggctctatggcttctgaggcggaaagaaccagctggggctctagggggtatccccacgcgccctgtagcggcgcattaagcgcggcgggtgtggtggttacgcgcagcgtgaccgctacacttgccagcgccctagcgcccgctcctttcgctttcttcccttcctttctcgccacgttcgccggctttccccgtcaagctctaaatcggggcatccctttagggttccgatttagtgctttacggcacctcgaccccaaaaaacttgattagggtgatggttcacgtagtgggccatcgccctgatagacggtttttcgccctttgacgttggagtccacgttctttaatagtggactcttgttccaaactggaacaacactcaaccctatctcggtctattcttttgatttataagggattttggggatttcggcctattggttaaaaaatgagctgatttaacaaaaatttaacgcgaattaattctgtggaatgtgtgtcagttagggtgtggaaagtccccaggctccccaggcaggcagaagtatgcaaagcatgcatctcaattagtcagcaaccaggtgtggaaagtccccaggctccccagcaggcagaagtatgcaaagcatgcatctcaattagtcagcaaccatagtcccgcccctaactccgcccatcccgcccctaactccgcccagttccgcccattctccgccccatggctgactaattttttttatttatgcagaggccgaggccgcctctgcctctgagctattccagaagtagtgaggaggcttttttggaggcctaggcttttgcaaaaagctcccgggagcttgtatatccattttcggatctgatcagcacgtgatgaaaaagcctgaactcaccgcgacgtctgtcgagaagtttctgatcgaaaagttcgacagcgtctccgacctgatgcagctctcggagggcgaagaatctcgtgctttcagcttcgatgtaggagggcgtggatatgtcctgcgggtaaatagctgcgccgatggtttctacaaagatcgttatgtttatcggcactttgcatcggccgcgctcccgattccggaagtgcttgacattggggaattcagcgagagcctgacctattgcatctcccgccgtgcacagggtgtcacgttgcaagacctgcctgaaaccgaactgcccgctgttctgcagccggtcgcggaggccatggatgcgatcgctgcggccgatcttagccagacgagcgggttcggcccattcggaccgcaaggaatcggtcaatacactacatggcgtgatttcatatgcgcgattgctgatccccatgtgtatcactggcaaactgtgatggacgacaccgtcagtgcgtccgtcgcgcaggctctcgatgagctgatgctttgggccgaggactgccccgaagtccggcacctcgtgcacgcggatttcggctccaacaatgtcctgacggacaatggccgcataacagcggtcattgactggagcgaggcgatgttcggggattcccaatacgaggtcgccaacatcttcttctggaggccgtggttggcttgtatggagcagcagacgcgctacttcgagcggaggcatccggagcttgcaggatcgccgcggctccgggcgtatatgctccgcattggtcttgaccaactctatcagagcttggttgacggcaatttcgatgatgcagcttgggcgcagggtcgatgcgacgcaatcgtccgatccggagccgggactgtcgggcgtacacaaatcgcccgcagaagcgcggccgtctggaccgatggctgtgtagaagtactcgccgatagtggaaaccgacgccccagcactcgtccgagggcaaaggaatagcacgtgctacgagatttcgattccaccgccgccttctatgaaaggttgggcttcggaatcgttttccgggacgccggctggatgatcctccagcgcggggatctcatgctggagttcttcgcccaccccaacttgtttattgcagcttataatggttacaaataaagcaatagcatcacaaatttcacaaataaagcatttttttcactgcattctagttgtggtttgtccaaactcatcaatgtatcttatcatgtctgtataccgtcgacctctagctagagcttggcgtaatcatggtcatagctgtttcctgtgtgaaattgttatccgctcacaattccacacaacatacgagccggaagcataaagtgtaaagcctggggtgcctaatgagtgagctaactcacattaattgcgttgcgctcactgcccgctttccagtcgggaaacctgtcgtgccagctgcattaatgaatcggccaacgcgcggggagaggcggtttgcgtattgggcgctcttccgcttcctcgctcactgactcgctgcgctcggtcgttcggctgcggcgagcggtatcagctcactcaaaggcggtaatacggttatccacagaatcaggggataacgcaggaaagaacatgtgagcaaaaggccagcaaaaggccaggaaccgtaaaaaggccgcgttgctggcgtttttccataggctccgcccccctgacgagcatcacaaaaatcgacgctcaagtcagaggtggcgaaacccgacaggactataaagataccaggcgtttccccctggaagctccctcgtgcgctctcctgttccgaccctgccgcttaccggatacctgtccgcctttctcccttcgggaagcgtggcgctttctcaatgctcacgctgtaggtatctcagttcggtgtaggtcgttcgctccaagctgggctgtgtgcacgaaccccccgttcagcccgaccgctgcgccttatccggtaactatcgtcttgagtccaacccggtaagacacgacttatcgccactggcagcagccactggtaacaggattagcagagcgaggtatgtaggcggtgctacagagttcttgaagtggtggcctaactacggctacactagaaggacagtatttggtatctgcgctctgctgaagccagttaccttcggaaaaagagttggtagctcttgatccggcaaacaaaccaccgctggtagcggtggtttttttgtttgcaagcagcagattacgcgcagaaaaaaaggatctcaagaagatcctttgatcttttctacggggtctgacgctcagtggaacgaaaactcacgttaagggattttggtcatgagattatcaaaaaggatcttcacctagatccttttaaattaaaaatgaagttttaaatcaatctaaagtatatatgagtaaacttggtctgacagttaccaatgcttaatcagtgaggcacctatctcagcgatctgtctatttcgttcatccatagttgcctgactccccgtcgtgtagataactacgatacgggagggcttaccatctggccccagtgctgcaatgataccgcgagacccacgctcaccggctccagatttatcagcaataaaccagccagccggaagggccgagcgcagaagtggtcctgcaactttatccgcctccatccagtctattaattgttgccgggaagctagagtaagtagttcgccagttaatagtttgcgcaacgttgttgccattgctacaggcatcgtggtgtcacgctcgtcgtttggtatggcttcattcagctccggttcccaacgatcaaggcgagttacatgatcccccatgttgtgcaaaaaagcggttagctccttcggtcctccgatcgttgtcagaagtaagttggccgcagtgttatcactcatggttatggcagcactgcataattctcttactgtcatgccatccgtaagatgcttttctgtgactggtgagtactcaaccaagtcattctgagaatagtgtatgcggcgaccgagttgctcttgcccggcgtcaatacgggataataccgcgccacatagcagaactttaaaagtgctcatcattggaaaacgttcttcggggcgaaaactctcaaggatcttaccgctgttgagatccagttcgatgtaacccactcgtgcacccaactgatcttcagcatcttttactttcaccagcgtttctgggtgagcaaaaacaggaaggcaaaatgccgcaaaaaagggaataagggcgacacggaaatgttgaatactcatactcttcctttttcaatattattgaagcatttatcagggttattgtctcatgagcggatacatatttgaatgtatttagaaaaataaacaaataggggttccgcgcacatttccccgaaaagtgccacctgacgtc

SEQ ID NO: 23 - protein, 206 aa, Artificial Sequence
  amino acid sequence of sortase A from Staphylococcus aureus
MKKWTNRLMTIAGVVLILVAAYLFAKPHIDNYLHDKDKDEKIEQYDKNVKEQASKDKKQQAKPQIPKDKSKVAGYIEIPDADIKEPVYPGPATPEQLNRGVSFAEENESLDDQNISIAGHTFIDRPNYQFTNLKAAKKGSMVYFKVGNETRKYKMTSIRDVKPTDVGVLDEQKGKDKQLTLITCDDYNEKTGVWEKRKIFVATEVK

SEQ ID NO: 24 - DNA, 621 bp, Artificial Sequence
  Nucleotide sequence encoding for SEQ ID NO 23
atgaaaaaatggacaaatcgattaatgacaatcgctggtgtggtacttatcctagtggcagcatatttgtttgctaaaccacatatcgataattatcttcacgataaagataaagatgaaaagattgaacaatatgataaaaatgtaaaagaacaggcgagtaaagataaaaagcagcaagctaaacctcaaattccgaaagataaatcgaaagtggcaggctatattgaaattccagatgctgatattaaagaaccagtatatccaggaccagcaacacctgaacaattaaatagaggtgtaagctttgcagaagaaaatgaatcactagatgatcaaaatatttcaattgcaggacacactttcattgaccgtccgaactatcaatttacaaatcttaaagcagccaaaaaaggtagtatggtgtactttaaagttggtaatgaaacacgtaagtataaaatgacaagtataagagatgttaagcctacagatgtaggagttctagatgaacaaaaaggtaaagataaacaattaacattaattacttgtgatgattacaatgaaaagacaggcgtttgggaaaaacgtaaaatctttgtagctacagaagtcaaataa

SEQ ID NO: 25 - DNA, 465 bp, Artificial Sequence
  coding region for a 6xHis tagged version of Staphylococcus aureus sortase A (aa60-205)
atgcaagctaaacctcaaattccgaaagataaatcgaaagtggcaggctatattgaaattccagatgctgatattaaagaaccagtatatccaggaccagcaacacctgaacaattaaatagaggtgtaagctttgcagaagaaaatgaatcactagatgatcaaaatatttcaattgcaggacacactttcattgaccgtccgaactatcaatttacaaatcttaaagcagccaaaaaaggtagtatggtgtactttaaagttggtaatgaaacacgtaagtataaaatgacaagtataagagatgttaagcctacagatgtaggagttctagatgaacaaaaaggtaaagataaacaattaacattaattacttgtgatgattacaatgaaaagacaggcgtttgggaaaaacgtaaaatctttgtagctacagaagtcaaacaccatcaccatcaccattaa

SEQ ID NO: 26 - protein, 154 aa, Artificial Sequence
  Amino acid sequence translated from SEQ ID NO 25
MQAKPQIPKDKSKVAGYIEIPDADIKEPVYPGPATPEQLNRGVSFAEENESLDDQNISIAGHTFIDRPNYQFTNLKAAKKGSMVYFKVGNETRKYKMTSIRDVKPTDVGVLDEQKGKDKQLTLITCDDYNEKTGVWEKRKIFVATEVKHHHHHH

SEQ ID NO: 27 - DNA, 1401 bp, Artificial Sequence
  Nucleotide sequence of mAb Ac10 Heavy Chain
atgaattttggactgaggctgattttcctggtgctgaccctgaaaggcgtccagtgtcagatccagctgcagcagtctggccccgaggtcgtgaaacctggcgcctccgtgaagatctcctgcaaggcctccggctacaccttcaccgactactacatcacctgggtcaagcagaagcccggccagggcctggaatggatcggctggatctatcccggctccggcaacaccaagtacaacgagaagttcaagggcaaggccaccctgaccgtggacacctcctcttccaccgccttcatgcagctgtcctccctgacctccgaggataccgccgtgtacttctgcgccaactacggcaactattggttcgcctactggggccagggcacacaagtgaccgtgtctgctgctagcaccaagggcccatcggtcttccccctggcaccctcctccaagagcacctctgggggcacagcagccctgggctgcctggtcaaggactacttccccgaaccggtgacggtgtcgtggaactcaggcgccctgaccagcggcgtgcacaccttcccggctgtcctacagtcctcaggactctactccctcagcagcgtggtgaccgtgccctccagcagcttgggcacccagacctacatctgcaacgtgaatcacaagcccagcaacaccaaggtggacaagaaagttgagcccaaatcttgtgacaaaactcacacatgcccaccgtgcccagcacctgaactcctggggggaccgtcagtcttcctcttccccccaaaacccaaggacaccctcatgatctcccggacccctgaggtcacatgcgtggtggtggacgtgagccacgaagaccctgaggtcaagttcaactggtacgtggacggcgtggaggtgcataatgccaagacaaagccgcgggaggagcagtacaacagcacgtaccgtgtggtcagcgtcctcaccgtcctgcaccaggactggctgaatggcaaggagtacaagtgcaaggtctccaacaaagccctcccagcccccatcgagaaaaccatctccaaagccaaagggcagccccgagaaccacaggtgtacaccctgcccccatcccgggatgagctgaccaagaaccaggtcagcctgacctgcctggtcaaaggcttctatcccagcgacatcgccgtggagtgggagagcaatgggcagccggagaacaactacaagaccacgcctcccgtgctggactccgacggctccttcttcctctacagcaagctcaccgtggacaagagcaggtggcagcaggggaacgtcttctcatgctccgtgatgcatgaggctctgcacaaccactacacacagaagagcctctccctgtctccgggtaaatag

SEQ ID NO: 28 - protein, 466 aa, Artificial Sequence
  AMINO ACID SEQUENCE OF MAB AC10 HEAVY CHAIN
MNFGLRLIFLVLTLKGVQCQIQLQQSGPEVVKPGASVKISCKASGYTFTDYYITWVKQKPGQGLEWIGWIYPGSGNTKYNEKFKGKATLTVDTSSSTAFMQLSSLTSEDTAVYFCANYGNYWFAYWGQGTQVTVSAASTKGPSVFPLAPSSKSTSGGTAALGCLVKDYFPEPVTVSWNSGALTSGVHTFPAVLQSSGLYSLSSVVTVPSSSLGTQTYICNVNHKPSNTKVDKKVEPKSCDKTHTCPPCPAPELLGGPSVFLFPPKPKDTLMISRTPEVTCVVVDVSHEDPEVKFNWYVDGVEVHNAKTKPREEQYNSTYRVVSVLTVLHQDWLNGKEYKCKVSNKALPAPIEKTISKAKGQPREPQVYTLPPSRDELTKNQVSLTCLVKGFYPSDIAVEWESNGQPENNYKTTPPVLDSDGSFFLYSKLTVDKSRWQQGNVFSCSVMHEALHNHYTQKSLSLSPGK

SEQ ID NO: 29 - DNA, 714 bp, Artificial Sequence
  Nucleotide sequence of mAb Ac10 Light Chain
atgaattttggactgaggctgattttcctggtgctgaccctgaaaggcgtccagtgtgacattgtgctgacccaatctccagcttctttggctgtgtctctagggcagagggccaccatctcctgcaaggccagccaaagtgttgattttgatggtgatagttatatgaactggtaccaacagaaaccaggacagccacccaaagtcctcatctatgctgcatccaatctagaatctgggatcccagccaggtttagtggcagtgggtctgggacagacttcaccctcaacatccatcctgtggaggaggaggatgctgcaacctattactgtcagcaaagtaatgaggatccgtggacgttcggtggaggcaccaagctggaaatcaaacgtacggtggctgcaccatctgtcttcatcttcccgccatctgatgagcagttgaaatctggaactgcctctgttgtgtgcctgctgaataacttctatcccagagaggccaaagtacagtggaaggtggataacgccctccaatcgggtaactcccaggagagtgtcacagagcaggacagcaaggacagcacctacagcctcagcagcaccctgacgctgagcaaagcagactacgagaaacacaaagtctacgcctgcgaagtcacccatcagggcctgagctcgcccgtcacaaagagcttcaacaggggagagtgttag

SEQ ID NO: 30 - protein, 237 aa, Artificial Sequence
  Amino acid sequence of mAb Ac10 Light Chain
MNFGLRLIFLVLTLKGVQCDIVLTQSPASLAVSLGQRATISCKASQSVDFDGDSYMNWYQQKPGQPPKVLIYAASNLESGIPARFSGSGSGTDFTLNIHPVEEEDAATYYCQQSNEDPWTFGGGTKLEIKRTVAAPSVFIFPPSDEQLKSGTASVVCLLNNFYPREAKVQWKVDNALQSGNSQESVTEQDSKDSTYSLSSTLTLSKADYEKHKVYACEVTHQGLSSPVTKSFNRGEC

SEQ ID NO: 31 - DNA, 1422 bp, Artificial Sequence
  Nucleotide sequence of Trastuzumab Heavy Chain
atgaaaaaaaacattgcctttctgctggcctccatgttcgtgttctctatcgccacaaacgcttacgctgaagtccagctggtcgaatctggtggtggcctggtccagcctggtggatcactgagactgtcctgtgctgcttctggtttcaacatcaaggacacctacatccattgggtcagacaggcacctggcaagggactggaatgggtcgcccgaatctaccctacaaacggctacactcgctacgccgactccgtcaagggacgctttaccatctccgccgacacctctaaaaacaccgcctacctgcagatgaatagtctgagggccgaggatactgctgtgtactactgctcacgatggggaggcgacggcttttacgctatggattactggggacagggaactctggtcactgtgtctagcgctagcaccaagggcccatcggtcttccccctggcaccctcctccaagagcacctctgggggcacagcagccctgggctgcctggtcaaggactacttccccgaaccggtgacggtgtcgtggaactcaggcgccctgaccagcggcgtgcacaccttcccggctgtcctacagtcctcaggactctactccctcagcagcgtggtgaccgtgccctccagcagcttgggcacccagacctacatctgcaacgtgaatcacaagcccagcaacaccaaggtggacaagaaagttgagcccaaatcttgtgacaaaactcacacatgcccaccgtgcccagcacctgaactcctggggggaccgtcagtcttcctcttccccccaaaacccaaggacaccctcatgatctcccggacccctgaggtcacatgcgtggtggtggacgtgagccacgaagaccctgaggtcaagttcaactggtacgtggacggcgtggaggtgcataatgccaagacaaagccgcgggaggagcagtacaacagcacgtaccgtgtggtcagcgtcctcaccgtcctgcaccaggactggctgaatggcaaggagtacaagtgcaaggtctccaacaaagccctcccagcccccatcgagaaaaccatctccaaagccaaagggcagccccgagaaccacaggtgtacaccctgcccccatcccgggatgagctgaccaagaaccaggtcagcctgacctgcctggtcaaaggcttctatcccagcgacatcgccgtggagtgggagagcaatgggcagccggagaacaactacaagaccacgcctcccgtgctggactccgacggctccttcttcctctacagcaagctcaccgtggacaagagcaggtggcagcaggggaacgtcttctcatgctccgtgatgcatgaggctctgcacaaccactacacacagaagagcctctccctgtctccgggtaaatag

SEQ ID NO: 32 - protein, 473 aa, Artificial Sequence
  Amino acid sequence of Trastuzumab Heavy Chain
MKKNIAFLLASMFVFSIATNAYAEVQLVESGGGLVQPGGSLRLSCAASGFNIKDTYIHWVRQAPGKGLEWVARIYPTNGYTRYADSVKGRFTISADTSKNTAYLQMNSLRAEDTAVYYCSRWGGDGFYAMDYWGQGTLVTVSSASTKGPSVFPLAPSSKSTSGGTAALGCLVKDYFPEPVTVSWNSGALTSGVHTFPAVLQSSGLYSLSSVVTVPSSSLGTQTYICNVNHKPSNTKVDKKVEPKSCDKTHTCPPCPAPELLGGPSVFLFPPKPKDTLMISRTPEVTCVVVDVSHEDPEVKFNWYVDGVEVHNAKTKPREEQYNSTYRVVSVLTVLHQDWLNGKEYKCKVSNKALPAPIEKTISKAKGQPREPQVYTLPPSRDELTKNQVSLTCLVKGFYPSDIAVEWESNGQPENNYKTTPPVLDSDGSFFLYSKLTVDKSRWQQGNVFSCSVMHEALHNHYTQKSLSLSPGK

SEQ ID NO: 33 - DNA, 1491 bp, Artificial Sequence
  Nucleotide sequence of Trastuzumab Heavy Chain with C-terminal GS peptide spacer, LPETG sortase A recognition motif and additional 6x-His and strep-II affinity purification tags
atgaaaaaaaacattgcctttctgctggcctccatgttcgtgttctctatcgccacaaacgcttacgctgaagtccagctggtcgaatctggtggtggcctggtccagcctggtggatcactgagactgtcctgtgctgcttctggtttcaacatcaaggacacctacatccattgggtcagacaggcacctggcaagggactggaatgggtcgcccgaatctaccctacaaacggctacactcgctacgccgactccgtcaagggacgctttaccatctccgccgacacctctaaaaacaccgcctacctgcagatgaatagtctgagggccgaggatactgctgtgtactactgctcacgatggggaggcgacggcttttacgctatggattactggggacagggaactctggtcactgtgtctagcgctagcaccaagggcccatcggtcttccccctggcaccctcctccaagagcacctctgggggcacagcagccctgggctgcctggtcaaggactacttccccgaaccggtgacggtgtcgtggaactcaggcgccctgaccagcggcgtgcacaccttcccggctgtcctacagtcctcaggactctactccctcagcagcgtggtgaccgtgccctccagcagcttgggcacccagacctacatctgcaacgtgaatcacaagcccagcaacaccaaggtggacaagaaagttgagcccaaatcttgtgacaaaactcacacatgcccaccgtgcccagcacctgaactcctggggggaccgtcagtcttcctcttccccccaaaacccaaggacaccctcatgatctcccggacccctgaggtcacatgcgtggtggtggacgtgagccacgaagaccctgaggtcaagttcaactggtacgtggacggcgtggaggtgcataatgccaagacaaagccgcgggaggagcagtacaacagcacgtaccgtgtggtcagcgtcctcaccgtcctgcaccaggactggctgaatggcaaggagtacaagtgcaaggtctccaacaaagccctcccagcccccatcgagaaaaccatctccaaagccaaagggcagccccgagaaccacaggtgtacaccctgcccccatcccgggatgagctgaccaagaaccaggtcagcctgacctgcctggtcaaaggcttctatcccagcgacatcgccgtggagtgggagagcaatgggcagccggagaacaactacaagaccacgcctcccgtgctggactccgacggctccttcttcctctacagcaagctcaccgtggacaagagcaggtggcagcaggggaacgtcttctcatgctccgtgatgcatgaggctctgcacaaccactacacacagaagagcctctccctgtctccgggtaaaggatccctgcccgagaccggcggacaccatcaccatcaccatggctggagccacccccagttcgagaagtag

SEQ ID NO: 34 - protein, 496 aa, Artificial Sequence
  Amino acid sequence of Trastuzumab Heavy Chain with C-terminal GS peptide spacer, LPETG sortase A recognition motif and additional 6x-His and strep-II affinity purification tags
MKKNIAFLLASMFVFSIATNAYAEVQLVESGGGLVQPGGSLRLSCAASGFNIKDTYIHWVRQAPGKGLEWVARIYPTNGYTRYADSVKGRFTISADTSKNTAYLQMNSLRAEDTAVYYCSRWGGDGFYAMDYWGQGTLVTVSSASTKGPSVFPLAPSSKSTSGGTAALGCLVKDYFPEPVTVSWNSGALTSGVHTFPAVLQSSGLYSLSSVVTVPSSSLGTQTYICNVNHKPSNTKVDKKVEPKSCDKTHTCPPCPAPELLGGPSVFLFPPKPKDTLMISRTPEVTCVVVDVSHEDPEVKFNWYVDGVEVHNAKTKPREEQYNSTYRVVSVLTVLHQDWLNGKEYKCKVSNKALPAPIEKTISKAKGQPREPQVYTLPPSRDELTKNQVSLTCLVKGFYPSDIAVEWESNGQPENNYKTTPPVLDSDGSFFLYSKLTVDKSRWQQGNVFSCSVMHEALHNHYTQKSLSLSPGKGSLPETGGHHHHHHGWSHPQFEK

SEQ ID NO: 35 - DNA, 714 bp, Artificial Sequence
  Nucleotide sequence of Trastuzumab Light Chain
atgaaaaaaaacattgcctttctgctggcctccatgttcgtgttctctatcgccacaaatgcttatgccgacatccagatgacacagtctccctcttccctgtccgcttctgtgggcgatcgagtgacaatcacctgtagggctagtcaggatgtgaatactgctgttgcttggtaccagcagaaaccaggaaaagcccctaaactgctgatctactctgcctcattcctgtactctggggtgccttctcgattcagtggttctagatctggcaccgatttcacactgaccatttcttcactgcaacctgaggattttgccacctactactgtcagcagcactacacaacacctcccacatttggccagggcacaaaagtggagatcaaacgtacggtggctgcaccatctgtcttcatcttcccgccatctgatgagcagttgaaatctggaactgcctctgttgtgtgcctgctgaataacttctatcccagagaggccaaagtacagtggaaggtggataacgccctccaatcgggtaactcccaggagagtgtcacagagcaggacagcaaggacagcacctacagcctcagcagcaccctgacgctgagcaaagcagactacgagaaacacaaagtctacgcctgcgaagtcacccatcagggcctgagctcgcccgtcacaaagagcttcaacaggggagagtgttag

SEQ ID NO: 36 - protein, 237 aa, Artificial Sequence
  Amino acid sequence of Trastuzumab Light Chain
MKKNIAFLLASMFVFSIATNAYADIQMTQSPSSLSASVGDRVTITCRASQDVNTAVAWYQQKPGKAPKLLIYSASFLYSGVPSRFSGSRSGTDFTLTISSLQPEDFATYYCQQHYTTPPTFGQGTKVEIKRTVAAPSVFIFPPSDEQLKSGTASVVCLLNNFYPREAKVQWKVDNALQSGNSQESVTEQDSKDSTYSLSSTLTLSKADYEKHKVYACEVTHQGLSSPVTKSFNRGEC

SEQ ID NO: 37 - DNA, 783 bp, Artificial Sequence
  Nucleotide sequence of Trastuzumab Light Chain with C-terminal GS peptide spacer, LPETG sortase A recognition motif and additional 6x-His and strep-II affinity purification tags
atgaaaaaaaacattgcctttctgctggcctccatgttcgtgttctctatcgccacaaatgcttatgccgacatccagatgacacagtctccctcttccctgtccgcttctgtgggcgatcgagtgacaatcacctgtagggctagtcaggatgtgaatactgctgttgcttggtaccagcagaaaccaggaaaagcccctaaactgctgatctactctgcctcattcctgtactctggggtgccttctcgattcagtggttctagatctggcaccgatttcacactgaccatttcttcactgcaacctgaggattttgccacctactactgtcagcagcactacacaacacctcccacatttggccagggcacaaaagtggagatcaaacgtacggtggctgcaccatctgtcttcatcttcccgccatctgatgagcagttgaaatctggaactgcctctgttgtgtgcctgctgaataacttctatcccagagaggccaaagtacagtggaaggtggataacgccctccaatcgggtaactcccaggagagtgtcacagagcaggacagcaaggacagcacctacagcctcagcagcaccctgacgctgagcaaagcagactacgagaaacacaaagtctacgcctgcgaagtcacccatcagggcctgagctcgcccgtcacaaagagcttcaacaggggagagtgtggatccctgcccgagaccggcggacaccatcaccatcaccatggctggagccacccccagttcgagaagtag

SEQ ID NO: 38 - protein, 260 aa, Artificial Sequence
  Amino acid sequence of Trastuzumab Light Chain with C-terminal GS peptide-spacer, LPETG sortase A recognition motif and additional 6x-His and strep-II affinity purification tags
MKKNIAFLLASMFVFSIATNAYADIQMTQSPSSLSASVGDRVTITCRASQDVNTAVAWYQQKPGKAPKLLIYSASFLYSGVPSRFSGSRSGTDFTLTISSLQPEDFATYYCQQHYTTPPTFGQGTKVEIKRTVAAPSVFIFPPSDEQLKSGTASVVCLLNNFYPREAKVQWKVDNALQSGNSQESVTEQDSKDSTYSLSSTLTLSKADYEKHKVYACEVTHQGLSSPVTKSFNRGECGSLPETGGHHHHHHGWSHPQFEK

SEQ ID NO: 39 - DNA, 1470 bp, Artificial Sequence
  Nucleotide sequence of mAb Ac10 Heavy Chain with C-terminal GS peptide-spacer, LPETG sortase A recognition motif and additional 6x-His and strep-II affinity purification tags
atgaattttggactgaggctgattttcctggtgctgaccctgaaaggcgtccagtgtcagatccagctgcagcagtctggccccgaggtcgtgaaacctggcgcctccgtgaagatctcctgcaaggcctccggctacaccttcaccgactactacatcacctgggtcaagcagaagcccggccagggcctggaatggatcggctggatctatcccggctccggcaacaccaagtacaacgagaagttcaagggcaaggccaccctgaccgtggacacctcctcttccaccgccttcatgcagctgtcctccctgacctccgaggataccgccgtgtacttctgcgccaactacggcaactattggttcgcctactggggccagggcacacaagtgaccgtgtctgctgctagcaccaagggcccatcggtcttccccctggcaccctcctccaagagcacctctgggggcacagcagccctgggctgcctggtcaaggactacttccccgaaccggtgacggtgtcgtggaactcaggcgccctgaccagcggcgtgcacaccttcccggctgtcctacagtcctcaggactctactccctcagcagcgtggtgaccgtgccctccagcagcttgggcacccagacctacatctgcaacgtgaatcacaagcccagcaacaccaaggtggacaagaaagttgagcccaaatcttgtgacaaaactcacacatgcccaccgtgcccagcacctgaactcctggggggaccgtcagtcttcctcttccccccaaaacccaaggacaccctcatgatctcccggacccctgaggtcacatgcgtggtggtggacgtgagccacgaagaccctgaggtcaagttcaactggtacgtggacggcgtggaggtgcataatgccaagacaaagccgcgggaggagcagtacaacagcacgtaccgtgtggtcagcgtcctcaccgtcctgcaccaggactggctgaatggcaaggagtacaagtgcaaggtctccaacaaagccctcccagcccccatcgagaaaaccatctccaaagccaaagggcagccccgagaaccacaggtgtacaccctgcccccatcccgggatgagctgaccaagaaccaggtcagcctgacctgcctggtcaaaggcttctatcccagcgacatcgccgtggagtgggagagcaatgggcagccggagaacaactacaagaccacgcctcccgtgctggactccgacggctccttcttcctctacagcaagctcaccgtggacaagagcaggtggcagcaggggaacgtcttctcatgctccgtgatgcatgaggctctgcacaaccactacacacagaagagcctctccctgtctccgggtaaaggatccctgcccgagaccggcggacaccatcaccatcaccatggctggagccacccccagttcgagaagtag

SEQ ID NO: 40 - protein, 489 aa, Artificial Sequence
  Amino acid sequence of mAb Ac10 Heavy Chain with C-terminal GS peptide-spacer, LPETG sortase A recognition motif and additional 6x-His and strep II affinity purification tags
MNFGLRLIFLVLTLKGVQCQIQLQQSGPEVVKPGASVKISCKASGYTFTDYYITWVKQKPGQGLEWIGWIYPGSGNTKYNEKFKGKATLTVDTSSSTAFMQLSSLTSEDTAVYFCANYGNYWFAYWGQGTQVTVSAASTKGPSVFPLAPSSKSTSGGTAALGCLVKDYFPEPVTVSWNSGALTSGVHTFPAVLQSSGLYSLSSVVTVPSSSLGTQTYICNVNHKPSNTKVDKKVEPKSCDKTHTCPPCPAPELLGGPSVFLFPPKPKDTLMISRTPEVTCVVVDVSHEDPEVKFNWYVDGVEVHNAKTKPREEQYNSTYRVVSVLTVLHQDWLNGKEYKCKVSNKALPAPIEKTISKAKGQPREPQVYTLPPSRDELTKNQVSLTCLVKGFYPSDIAVEWESNGQPENNYKTTPPVLDSDGSFFLYSKLTVDKSRWQQGNVFSCSVMHEALHNHYTQKSLSLSPGKGSLPETGGHHHHHHGWSHPQFEK

SEQ ID NO: 41 - DNA, 783 bp, Artificial Sequence
  Nucleotide sequence of mAb Ac10 Light Chain with C-terminal GS peptide-spacer, LPETG sortase A recognition motif and additional 6x-His and strep II affinity purification tags
atgaattttggactgaggctgattttcctggtgctgaccctgaaaggcgtccagtgtgacattgtgctgacccaatctccagcttctttggctgtgtctctagggcagagggccaccatctcctgcaaggccagccaaagtgttgattttgatggtgatagttatatgaactggtaccaacagaaaccaggacagccacccaaagtcctcatctatgctgcatccaatctagaatctgggatcccagccaggtttagtggcagtgggtctgggacagacttcaccctcaacatccatcctgtggaggaggaggatgctgcaacctattactgtcagcaaagtaatgaggatccgtggacgttcggtggaggcaccaagctggaaatcaaacgtacggtggctgcaccatctgtcttcatcttcccgccatctgatgagcagttgaaatctggaactgcctctgttgtgtgcctgctgaataacttctatcccagagaggccaaagtacagtggaaggtggataacgccctccaatcgggtaactcccaggagagtgtcacagagcaggacagcaaggacagcacctacagcctcagcagcaccctgacgctgagcaaagcagactacgagaaacacaaagtctacgcctgcgaagtcacccatcagggcctgagctcgcccgtcacaaagagcttcaacaggggagagtgtggatccctgcccgagaccggcggacaccatcaccatcaccatggctggagccacccccagttcgagaagtag

SEQ ID NO: 42 - protein, 260 aa, Artificial Sequence
  Amino acid sequence of mAb Ac10 Light Chain with C-terminal GS peptide-spacer, LPETG sortase A recognition motif and additional 6x-His and strep II affinity purification tags
MNFGLRLIFLVLTLKGVQCDIVLTQSPASLAVSLGQRATISCKASQSVDFDGDSYMNWYQQKPGQPPKVLIYAASNLESGIPARFSGSGSGTDFTLNIHPVEEEDAATYYCQQSNEDPWTFGGGTKLEIKRTVAAPSVFIFPPSDEQLKSGTASVVCLLNNFYPREAKVQWKVDNALQSGNSQESVTEQDSKDSTYSLSSTLTLSKADYEKHKVYACEVTHQGLSSPVTKSFNRGECGSLPETGGHHHHHHGWSHPQFEK

SEQ ID NO: 43 - DNA, 1443 bp, Artificial Sequence
  Nucleotide sequence of mAb Ac10 Heavy Chain with C-terminal LPETG sortase A recognition motif and strep II affinity purification tag
atgaattttggactgaggctgattttcctggtgctgaccctgaaaggcgtccagtgtcagatccagctgcagcagtctggccccgaggtcgtgaaacctggcgcctccgtgaagatctcctgcaaggcctccggctacaccttcaccgactactacatcacctgggtcaagcagaagcccggccagggcctggaatggatcggctggatctatcccggctccggcaacaccaagtacaacgagaagttcaagggcaaggccaccctgaccgtggacacctcctcttccaccgccttcatgcagctgtcctccctgacctccgaggataccgccgtgtacttctgcgccaactacggcaactattggttcgcctactggggccagggcacacaagtgaccgtgtctgctgctagcaccaagggcccatcggtcttccccctggcaccctcctccaagagcacctctgggggcacagcagccctgggctgcctggtcaaggactacttccccgaaccggtgacggtgtcgtggaactcaggcgccctgaccagcggcgtgcacaccttcccggctgtcctacagtcctcaggactctactccctcagcagcgtggtgaccgtgccctccagcagcttgggcacccagacctacatctgcaacgtgaatcacaagcccagcaacaccaaggtggacaagaaagttgagcccaaatcttgtgacaaaactcacacatgcccaccgtgcccagcacctgaactcctggggggaccgtcagtcttcctcttccccccaaaacccaaggacaccctcatgatctcccggacccctgaggtcacatgcgtggtggtggacgtgagccacgaagaccctgaggtcaagttcaactggtacgtggacggcgtggaggtgcataatgccaagacaaagccgcgggaggagcagtacaacagcacgtaccgtgtggtcagcgtcctcaccgtcctgcaccaggactggctgaatggcaaggagtacaagtgcaaggtctccaacaaagccctcccagcccccatcgagaaaaccatctccaaagccaaagggcagccccgagaaccacaggtgtacaccctgcccccatcccgggatgagctgaccaagaaccaggtcagcctgacctgcctggtcaaaggcttctatcccagcgacatcgccgtggagtgggagagcaatgggcagccggagaacaactacaagaccacgcctcccgtgctggactccgacggctccttcttcctctacagcaagctcaccgtggacaagagcaggtggcagcaggggaacgtcttctcatgctccgtgatgcatgaggctctgcacaaccactacacacagaagagcctctccctgtctccgggtaaactgcccgagaccggcggatggagccacccccagttcgagaagtag

SEQ ID NO: 44 - protein, 480 aa, Artificial Sequence
  Amino acid sequence of mAb Ac10 Heavy Chain with C-terminal LPETG sortase A recognition motif and strep-II affinity purification tag
MNFGLRLIFLVLTLKGVQCQIQLQQSGPEVVKPGASVKISCKASGYTFTDYYITWVKQKPGQGLEWIGWIYPGSGNTKYNEKFKGKATLTVDTSSSTAFMQLSSLTSEDTAVYFCANYGNYWFAYWGQGTQVTVSAASTKGPSVFPLAPSSKSTSGGTAALGCLVKDYFPEPVTVSWNSGALTSGVHTFPAVLQSSGLYSLSSVVTVPSSSLGTQTYICNVNHKPSNTKVDKKVEPKSCDKTHTCPPCPAPELLGGPSVFLFPPKPKDTLMISRTPEVTCVVVDVSHEDPEVKFNWYVDGVEVHNAKTKPREEQYNSTYRVVSVLTVLHQDWLNGKEYKCKVSNKALPAPIEKTISKAKGQPREPQVYTLPPSRDELTKNQVSLTCLVKGFYPSDIAVEWESNGQPENNYKTTPPVLDSDGSFFLYSKLTVDKSRWQQGNVFSCSVMHEALHNHYTQKSLSLSPGKLPETGGWSHPQFEK

SEQ ID NO: 45 - DNA, 756 bp, Artificial Sequence
  Nucleotide sequence of mAb Ac10 Light Chain with C-terminal LPETG sortase A recognition motif and strep-II affinity purification tag
atgaattttggactgaggctgattttcctggtgctgaccctgaaaggcgtccagtgtgacattgtgctgacccaatctccagcttctttggctgtgtctctagggcagagggccaccatctcctgcaaggccagccaaagtgttgattttgatggtgatagttatatgaactggtaccaacagaaaccaggacagccacccaaagtcctcatctatgctgcatccaatctagaatctgggatcccagccaggtttagtggcagtgggtctgggacagacttcaccctcaacatccatcctgtggaggaggaggatgctgcaacctattactgtcagcaaagtaatgaggatccgtggacgttcggtggaggcaccaagctggaaatcaaacgtacggtggctgcaccatctgtcttcatcttcccgccatctgatgagcagttgaaatctggaactgcctctgttgtgtgcctgctgaataacttctatcccagagaggccaaagtacagtggaaggtggataacgccctccaatcgggtaactcccaggagagtgtcacagagcaggacagcaaggacagcacctacagcctcagcagcaccctgacgctgagcaaagcagactacgagaaacacaaagtctacgcctgcgaagtcacccatcagggcctgagctcgcccgtcacaaagagcttcaacaggggagagtgtctgcccgagaccggcggatggagccacccccagttcgagaagtag

SEQ ID NO: 46 - protein, 251 aa, Artificial Sequence
  Amino acid sequence of mAb Ac10 Light Chain with C-terminal LPETG sortase A recognition motif and strep-II affinity purification tag
MNFGLRLIFLVLTLKGVQCDIVLTQSPASLAVSLGQRATISCKASQSVDFDGDSYMNWYQQKPGQPPKVLIYAASNLESGIPARFSGSGSGTDFTLNIHPVEEEDAATYYCQQSNEDPWTFGGGTKLEIKRTVAAPSVFIFPPSDEQLKSGTASVVCLLNNFYPREAKVQWKVDNALQSGNSQESVTEQDSKDSTYSLSSTLTLSKADYEKHKVYACEVTHQGLSSPVTKSFNRGECLPETGGWSHPQFEK

SEQ ID NO: 47 - DNA, 762 bp, Artificial Sequence
  Nucleotide sequence of mAb Ac10 Light Chain with C-terminal GS peptide-spacer, LPETG sortase A recognition motif and strep II affinity purification tag
atgaattttggactgaggctgattttcctggtgctgaccctgaaaggcgtccagtgtgacattgtgctgacccaatctccagcttctttggctgtgtctctagggcagagggccaccatctcctgcaaggccagccaaagtgttgattttgatggtgatagttatatgaactggtaccaacagaaaccaggacagccacccaaagtcctcatctatgctgcatccaatctagaatctgggatcccagccaggtttagtggcagtgggtctgggacagacttcaccctcaacatccatcctgtggaggaggaggatgctgcaacctattactgtcagcaaagtaatgaggatccgtggacgttcggtggaggcaccaagctggaaatcaaacgtacggtggctgcaccatctgtcttcatcttcccgccatctgatgagcagttgaaatctggaactgcctctgttgtgtgcctgctgaataacttctatcccagagaggccaaagtacagtggaaggtggataacgccctccaatcgggtaactcccaggagagtgtcacagagcaggacagcaaggacagcacctacagcctcagcagcaccctgacgctgagcaaagcagactacgagaaacacaaagtctacgcctgcgaagtcacccatcagggcctgagctcgcccgtcacaaagagcttcaacaggggagagtgtggatccctgcccgagaccggcggatggagccacccccagttcgagaagtag

SEQ ID NO: 48 - protein, 253 aa, Artificial Sequence
  Amino acid sequence of mAb Ac10 Light Chain with C-terminal GS peptide-spacer, LPETG sortase A recognition motif and strep II affinity purification tag
MNFGLRLIFLVLTLKGVQCDIVLTQSPASLAVSLGQRATISCKASQSVDFDGDSYMNWYQQKPGQPPKVLIYAASNLESGIPARFSGSGSGTDFTLNIHPVEEEDAATYYCQQSNEDPWTFGGGTKLEIKRTVAAPSVFIFPPSDEQLKSGTASVVCLLNNFYPREAKVQWKVDNALQSGNSQESVTEQDSKDSTYSLSSTLTLSKADYEKHKVYACEVTHQGLSSPVTKSFNRGECGSLPETGGWSHPQFEK

SEQ ID NO: 49 - DNA, 765 bp, Artificial Sequence
  Nucleotide sequence of mAb Ac10 Light Chain with C-terminal GGS peptide-spacer, LPETG sortase A recognition motif and strep II affinity purification tag
atgaattttggactgaggctgattttcctggtgctgaccctgaaaggcgtccagtgtgacattgtgctgacccaatctccagcttctttggctgtgtctctagggcagagggccaccatctcctgcaaggccagccaaagtgttgattttgatggtgatagttatatgaactggtaccaacagaaaccaggacagccacccaaagtcctcatctatgctgcatccaatctagaatctgggatcccagccaggtttagtggcagtgggtctgggacagacttcaccctcaacatccatcctgtggaggaggaggatgctgcaacctattactgtcagcaaagtaatgaggatccgtggacgttcggtggaggcaccaagctggaaatcaaacgtacggtggctgcaccatctgtcttcatcttcccgccatctgatgagcagttgaaatctggaactgcctctgttgtgtgcctgctgaataacttctatcccagagaggccaaagtacagtggaaggtggataacgccctccaatcgggtaactcccaggagagtgtcacagagcaggacagcaaggacagcacctacagcctcagcagcaccctgacgctgagcaaagcagactacgagaaacacaaagtctacgcctgcgaagtcacccatcagggcctgagctcgcccgtcacaaagagcttcaacaggggagagtgtggtggatccctgcccgagaccggcggatggagccacccccagttcgagaagtag

SEQ ID NO: 50 - protein, 254 aa, Artificial Sequence
  Amino acid sequence of mAb Ac10 Light Chain with C-terminal GGS peptide-spacer, LPETG sortase A recognition motif and strep II affinity purification tag
MNFGLRLIFLVLTLKGVQCDIVLTQSPASLAVSLGQRATISCKASQSVDFDGDSYMNWYQQKPGQPPKVLIYAASNLESGIPARFSGSGSGTDFTLNIHPVEEEDAATYYCQQSNEDPWTFGGGTKLEIKRTVAAPSVFIFPPSDEQLKSGTASVVCLLNNFYPREAKVQWKVDNALQSGNSQESVTEQDSKDSTYSLSSTLTLSKADYEKHKVYACEVTHQGLSSPVTKSFNRGECGGSLPETGGWSHPQFEK

SEQ ID NO: 51 - DNA, 768 bp, Artificial Sequence
  Nucleotide sequence of mAb Ac10 Light Chain with C-terminal GGGS peptide-spacer, LPETG sortase A recognition motif and strep II affinity purification tag
atgaattttggactgaggctgattttcctggtgctgaccctgaaaggcgtccagtgtgacattgtgctgacccaatctccagcttctttggctgtgtctctagggcagagggccaccatctcctgcaaggccagccaaagtgttgattttgatggtgatagttatatgaactggtaccaacagaaaccaggacagccacccaaagtcctcatctatgctgcatccaatctagaatctgggatcccagccaggtttagtggcagtgggtctgggacagacttcaccctcaacatccatcctgtggaggaggaggatgctgcaacctattactgtcagcaaagtaatgaggatccgtggacgttcggtggaggcaccaagctggaaatcaaacgtacggtggctgcaccatctgtcttcatcttcccgccatctgatgagcagttgaaatctggaactgcctctgttgtgtgcctgctgaataacttctatcccagagaggccaaagtacagtggaaggtggataacgccctccaatcgggtaactcccaggagagtgtcacagagcaggacagcaaggacagcacctacagcctcagcagcaccctgacgctgagcaaagcagactacgagaaacacaaagtctacgcctgcgaagtcacccatcagggcctgagctcgcccgtcacaaagagcttcaacaggggagagtgtgggggtggatccctgcccgagaccggcggatggagccacccccagttcgagaagtag

SEQ ID NO: 52 - protein, 255 aa, Artificial Sequence
  Amino acid sequence of mAb Ac10 Light Chain with C-terminal GGGS peptide-spacer, LPETG sortase A recognition motif and strep II affinity purification tag
MNFGLRLIFLVLTLKGVQCDIVLTQSPASLAVSLGQRATISCKASQSVDFDGDSYMNWYQQKPGQPPKVLIYAASNLESGIPARFSGSGSGTDFTLNIHPVEEEDAATYYCQQSNEDPWTFGGGTKLEIKRTVAAPSVFIFPPSDEQLKSGTASVVCLLNNFYPREAKVQWKVDNALQSGNSQESVTEQDSKDSTYSLSSTLTLSKADYEKHKVYACEVTHQGLSSPVTKSFNRGECGGGSLPETGGWSHPQFEK

SEQ ID NO: 53 - DNA, 771 bp, Artificial Sequence
  Nucleotide sequence of mAb Ac10 Light Chain with C-terminal GGGGS peptide-spacer, LPETG sortase A recognition motif and strep II affinity purification tag
atgaattttggactgaggctgattttcctggtgctgaccctgaaaggcgtccagtgtgacattgtgctgacccaatctccagcttctttggctgtgtctctagggcagagggccaccatctcctgcaaggccagccaaagtgttgattttgatggtgatagttatatgaactggtaccaacagaaaccaggacagccacccaaagtcctcatctatgctgcatccaatctagaatctgggatcccagccaggtttagtggcagtgggtctgggacagacttcaccctcaacatccatcctgtggaggaggaggatgctgcaacctattactgtcagcaaagtaatgaggatccgtggacgttcggtggaggcaccaagctggaaatcaaacgtacggtggctgcaccatctgtcttcatcttcccgccatctgatgagcagttgaaatctggaactgcctctgttgtgtgcctgctgaataacttctatcccagagaggccaaagtacagtggaaggtggataacgccctccaatcgggtaactcccaggagagtgtcacagagcaggacagcaaggacagcacctacagcctcagcagcaccctgacgctgagcaaagcagactacgagaaacacaaagtctacgcctgcgaagtcacccatcagggcctgagctcgcccgtcacaaagagcttcaacaggggagagtgtggagggggtggatccctgcccgagaccggcggatggagccacccccagttcgagaagtag

SEQ ID NO: 54 - protein, 256 aa, Artificial Sequence
  Amino acid sequence of mAb Ac10 Light Chain with C-terminal GGGGS peptide-spacer, LPETG sortase A recognition motif and strep II affinity purification tag
MNFGLRLIFLVLTLKGVQCDIVLTQSPASLAVSLGQRATISCKASQSVDFDGDSYMNWYQQKPGQPPKVLIYAASNLESGIPARFSGSGSGTDFTLNIHPVEEEDAATYYCQQSNEDPWTFGGGTKLEIKRTVAAPSVFIFPPSDEQLKSGTASVVCLLNNFYPREAKVQWKVDNALQSGNSQESVTEQDSKDSTYSLSSTLTLSKADYEKHKVYACEVTHQGLSSPVTKSFNRGECGGGGSLPETGGWSHPQFEK

SEQ ID NO: 55 - DNA, 1464 bp, Artificial Sequence
  Nucleotide sequence of Trastuzumab Heavy Chain with C-terminal LPETG Sortase tag and strep II affinity purification tag
atgaaaaaaaacattgcctttctgctggcctccatgttcgtgttctctatcgccacaaacgcttacgctgaagtccagctggtcgaatctggtggtggcctggtccagcctggtggatcactgagactgtcctgtgctgcttctggtttcaacatcaaggacacctacatccattgggtcagacaggcacctggcaagggactggaatgggtcgcccgaatctaccctacaaacggctacactcgctacgccgactccgtcaagggacgctttaccatctccgccgacacctctaaaaacaccgcctacctgcagatgaatagtctgagggccgaggatactgctgtgtactactgctcacgatggggaggcgacggcttttacgctatggattactggggacagggaactctggtcactgtgtctagcgctagcaccaagggcccatcggtcttccccctggcaccctcctccaagagcacctctgggggcacagcagccctgggctgcctggtcaaggactacttccccgaaccggtgacggtgtcgtggaactcaggcgccctgaccagcggcgtgcacaccttcccggctgtcctacagtcctcaggactctactccctcagcagcgtggtgaccgtgccctccagcagcttgggcacccagacctacatctgcaacgtgaatcacaagcccagcaacaccaaggtggacaagaaagttgagcccaaatcttgtgacaaaactcacacatgcccaccgtgcccagcacctgaactcctggggggaccgtcagtcttcctcttccccccaaaacccaaggacaccctcatgatctcccggacccctgaggtcacatgcgtggtggtggacgtgagccacgaagaccctgaggtcaagttcaactggtacgtggacggcgtggaggtgcataatgccaagacaaagccgcgggaggagcagtacaacagcacgtaccgtgtggtcagcgtcctcaccgtcctgcaccaggactggctgaatggcaaggagtacaagtgcaaggtctccaacaaagccctcccagcccccatcgagaaaaccatctccaaagccaaagggcagccccgagaaccacaggtgtacaccctgcccccatcccgggatgagctgaccaagaaccaggtcagcctgacctgcctggtcaaaggcttctatcccagcgacatcgccgtggagtgggagagcaatgggcagccggagaacaactacaagaccacgcctcccgtgctggactccgacggctccttcttcctctacagcaagctcaccgtggacaagagcaggtggcagcaggggaacgtcttctcatgctccgtgatgcatgaggctctgcacaaccactacacacagaagagcctctccctgtctccgggtaaactgcccgagaccggcggatggagccacccccagttcgagaagtag

SEQ ID NO: 56 - protein, 487 aa, Amino acid sequence of mAb Ac10 Heavy Chain with C-terminal LPETG Sortase tag and strep II affinity purification tag
MKKNIAFLLASMFVFSIATNAYAEVQLVESGGGLVQPGGSLRLSCAASGFNIKDTYIHWVRQAPGKGLEWVARIYPTNGYTRYADSVKGRFTISADTSKNTAYLQMNSLRAEDTAVYYCSRWGGDGFYAMDYWGQGTLVTVSSASTKGPSVFPLAPSSKSTSGGTAALGCLVKDYFPEPVTVSWNSGALTSGVHTFPAVLQSSGLYSLSSVVTVPSSSLGTQTYICNVNHKPSNTKVDKKVEPKSCDKTHTCPPCPAPELLGGPSVFLFPPKPKDTLMISRTPEVTCVVVDVSHEDPEVKFNWYVDGVEVHNAKTKPREEQYNSTYRVVSVLTVLHQDWLNGKEYKCKVSNKALPAPIEKTISKAKGQPREPQVYTLPPSRDELTKNQVSLTCLVKGFYPSDIAVEWESNGQPENNYKTTPPVLDSDGSFFLYSKLTVDKSRWQQGNVFSCSVMHEALHNHYTQKSLSLSPGKLPETGGWSHPQFEK

SEQ ID NO: 57 - DNA, 771 bp, Artificial Sequence
  Nucleotide sequence of Trastuzumab Light Chain with C-terminal GGGGS linker, LPETG Sortase tag and strep II affinity purification tag
atgaaaaaaaacattgcctttctgctggcctccatgttcgtgttctctatcgccacaaatgcttatgccgacatccagatgacacagtctccctcttccctgtccgcttctgtgggcgatcgagtgacaatcacctgtagggctagtcaggatgtgaatactgctgttgcttggtaccagcagaaaccaggaaaagcccctaaactgctgatctactctgcctcattcctgtactctggggtgccttctcgattcagtggttctagatctggcaccgatttcacactgaccatttcttcactgcaacctgaggattttgccacctactactgtcagcagcactacacaacacctcccacatttggccagggcacaaaagtggagatcaaacgtacggtggctgcaccatctgtcttcatcttcccgccatctgatgagcagttgaaatctggaactgcctctgttgtgtgcctgctgaataacttctatcccagagaggccaaagtacagtggaaggtggataacgccctccaatcgggtaactcccaggagagtgtcacagagcaggacagcaaggacagcacctacagcctcagcagcaccctgacgctgagcaaagcagactacgagaaacacaaagtctacgcctgcgaagtcacccatcagggcctgagctcgcccgtcacaaagagcttcaacaggggagagtgtggagggggtggatccctgcccgagaccggcggatggagccacccccagttcgagaagtag

SEQ ID NO: 58 - protein, 256 aa, Artificial Sequence
  Amino acid sequence of mAb Ac10 Light Chain with C-terminal GGGGS linker, LPETG Sortase tag and strep II affinity purification tag
MKKNIAFLLASMFVFSIATNAYADIQMTQSPSSLSASVGDRVTITCRASQDVNTAVAWYQQKPGKAPKLLIYSASFLYSGVPSRFSGSRSGTDFTLTISSLQPEDFATYYCQQHYTTPPTFGQGTKVEIKRTVAAPSVFIFPPSDEQLKSGTASVVCLLNNFYPREAKVQWKVDNALQSGNSQESVTEQDSKDSTYSLSSTLTLSKADYEKHKVYACEVTHQGLSSPVTKSFNRGECGGGGSLPETGGWSHPQFEK